European Patent Specification EP 3 493 829 B1, published April 17, 2024. Title: Compositions and Methods For Stroke Prevention in Pediatric Sickle Cell Anemia Patients. Applicant: Yale University Braddock, Demetrios. The sequence listing filed with the application follows.

SEQUENCE LISTING (76 sequences)

SEQ ID NO: 1 - protein, 925 aa, Homo sapiens
MERDGCAGGGSRGGEGGRAPREGPAGNGRDRGRSHAAEAPGDPQAAASLLAPMDVGEEPLEKAARARTAKDPNTYKVLSLVLSVCVLTTILGCIFGLKPSCAKEVKSCKGRCFERTFGNCRCDAACVELGNCCLDYQETCIEPEHIWTCNKFRCGEKRLTRSLCACSDDCKDKGDCCINYSSVCQGEKSWVEEPCESINEPQCPAGFETPPTLLFSLDGFRAEYLHTWGGLLPVISKLKKCGTYTKNMRPVYPTKTFPNHYSIVTGLYPESHGIIDNKMYDPKMNASFSLKSKEKFNPEWYKGEPIWVTAKYQGLKSGTFFWPGSDVEINGIFPDIYKMYNGSVPFEERILAVLQWLQLPKDERPHFYTLYLEEPDSSGHSYGPVSSEVIKALQRVDGMVGMLMDGLKELNLHRCLNLILISDHGMEQGSCKKYIYLNKYLGDVKNIKVIYGPAARLRPSDVPDKYYSFNYEGIARNLSCREPNQHFKPYLKHFLPKRLHFAKSDRIEPLTFYLDPQWQLALNPSERKYCGSGFHGSDNVFSNMQALFVGYGPGFKHGIEADTFENIEVYNLMCDLLNLTPAPNNGTHGSLNHLLKNPVYTPKHPKEVHPLVQCPFTRNPRDNLGCSCNPSILPIEDFQTQFNLTVAEEKIIKHETLPYGRPRVLQKENTICLLSQHQFMSGYSQDILMPLWTSYTVDRNDSFSTEDFSNCLYQDFRIPLSPVHKCSFYKNNTKVSYGFLSPPQLNKNSSGIYSEALLTTNIVPMYQSFQVIWRYFHDTLLRKYAEERNGVNVVSGPVFDFDYDGRCDSLENLRQKRRVIRNQEILIPTHFFIVLTSCKDTSQTPLHCENLDTLAFILPHRTDNSESCVHGKHDSSWVEELLMLHRARITDVEHITGLSFYQQRKEPVSDILKLKTHLPTFSQED

SEQ ID NO: 2 - protein, 888 aa, Homo sapiens
MARRSSFQSCQIISLFTFAVGVNICLGFTAHRIKRAEGWEEGPPTVLSDSPWTNISGSCKGRCFELQEAGPPDCRCDNLCKSYTSCCHDFDELCLKTARGWECTKDRCGEVRNEENACHCSEDCLARGDCCTNYQVVCKGESHWVDDDCEEIKAAECPAGFVRPPLIIFSVDGFRASYMKKGSKVMPNIEKLRSCGTHSPYMRPVYPTKTFPNLYTLATGLYPESHGIVGNSMYDPVFDATFHLRGREKFNHRWWGGQPLWITATKQGVKAGTFFWSVVIPHERRILTILQWLTLPDHERPSVYAFYSEQPDFSGHKYGPFGPEMTNPLREIDKIVGQLMDGLKQLKLHRCVNVIFVGDHGMEDVTCDRTEFLSNYLTNVDDITLVPGTLGRIRSKFSNNAKYDPKAIIANLTCKKPDQHFKPYLKQHLPKRLHYANNRRIEDIHLLVERRWHVARKPLDVYKKPSGKCFFQGDHGFDNKVNSMQTVFVGYGSTFKYKTKVPPFENIELYNVMCDLLGLKPAPNNGTHGSLNHLLRTNTFRPTMPEEVTRPNYPGIMYLQSDFDLGCTCDDKVEPKNKLDELNKRLHTKGSTEAETRKFRGSRNENKENINGNFEPRKERHLLYGRPAVLYRTRYDILYHTDFESGYSEIFLMPLWTSYTVSKQAEVSSVPDHLTSCVRPDVRVSPSFSQNCLAYKNDKQMSYGFLFPPYLSSSPEAKYDAFLVTNMVPMYPAFKRVWNYFQRVLVKKYASERNGVNVISGPIFDYDYDGLHDTEDKIKQYVEGSSIPVPTHYYSIITSCLDFTQPADKCDGPLSVSSFILPHRPDNEESCNSSEDESKWVEELMKMHTARVRDIEHLTSLDFFRKTSRSYPEILTLKTYLHTYESEI

SEQ ID NO: 3 - protein, 1 aa, Artificial Sequence
  chemically synthesized
  REPEAT (1)..(1): sequence can be repeated 1-15 times
D

SEQ ID NO: 4 - protein, 3 aa, Artificial Sequence
  chemically synthesized
  REPEAT (1)..(3): sequence can be repeated 1-10 times
DSS

SEQ ID NO: 5 - protein, 3 aa, Artificial Sequence
  chemically synsthesized
  REPEAT (1)..(3): sequence can be repeated 1-10 times
ESS

SEQ ID NO: 6 - protein, 3 aa, Artificial Sequence
  chemically synthesized
  REPEAT (1)..(3): sequence can be repeated 1-10 times
RQQ

SEQ ID NO: 7 - protein, 2 aa, Artificial Sequence
  chemically synthesized
  REPEAT (1)..(2): sequence can be repeated 1-10 times
KR

SEQ ID NO: 8 - protein, 1 aa, Artificial Sequence
  chemically synthesized
  REPEAT (1)..(1): sequence can be repeated 1-15 times
R

SEQ ID NO: 9 - protein, 16 aa, Artificial Sequence
  chemically synthesized
DSSSEEKFLRRIGRFG

SEQ ID NO: 10 - protein, 12 aa, Artificial Sequence
  chemically synthesized
EEEEEEEPRGDT

SEQ ID NO: 11 - protein, 12 aa, Artificial Sequence
  chemically synthesized
APWHLSSQYSRT

SEQ ID NO: 12 - protein, 12 aa, Artificial Sequence
  chemically synthesized
STLPIPHEFSRE

SEQ ID NO: 13 - protein, 12 aa, Artificial Sequence
  chemically synthesized
VTKHLNQISQSY

SEQ ID NO: 14 - protein, 1 aa, Artificial Sequence
  chemically synthesized
  REPEAT (1)..(1): sequence can be repeated 1-15 times
E

SEQ ID NO: 15 - protein, 925 aa, Artificial Sequence
  ENPP121
MERDGCAGGGSRGGEGGRAPREGPAGNGRDRGRSHAAEAPGDPQAAASLLAPMDVGEEPLEKAARARTAKDPNTYKIISLFTFAVGVNICLGFTAGLKPSCAKEVKSCKGRCFERTFGNCRCDAACVELGNCCLDYQETCIEPEHIWTCNKFRCGEKRLTRSLCACSDDCKDKGDCCINYSSVCQGEKSWVEEPCESINEPQCPAGFETPPTLLFSLDGFRAEYLHTWGGLLPVISKLKKCGTYTKNMRPVYPTKTFPNHYSIVTGLYPESHGIIDNKMYDPKMNASFSLKSKEKFNPEWYKGEPIWVTAKYQGLKSGTFFWPGSDVEINGIFPDIYKMYNGSVPFEERILAVLQWLQLPKDERPHFYTLYLEEPDSSGHSYGPVSSEVIKALQRVDGMVGMLMDGLKELNLHRCLNLILISDHGMEQGSCKKYIYLNKYLGDVKNIKVIYGPAARLRPSDVPDKYYSFNYEGIARNLSCREPNQHFKPYLKHFLPKRLHFAKSDRIEPLTFYLDPQWQLALNPSERKYCGSGFHGSDNVFSNMQALFVGYGPGFKHGIEADTFENIEVYNLMCDLLNLTPAPNNGTHGSLNHLLKNPVYTPKHPKEVHPLVQCPFTRNPRDNLGCSCNPSILPIEDFQTQFNLTVAEEKIIKHETLPYGRPRVLQKENTICLLSQHQFMSGYSQDILMPLWTSYTVDRNDSFSTEDFSNCLYQDFRIPLSPVHKCSFYKNNTKVSYGFLSPPQLNKNSSGIYSEALLTTNIVPMYQSFQVIWRYFHDTLLRKYAEERNGVNVVSGPVFDFDYDGRCDSLENLRQKRRVIRNQEILIPTHFFIVLTSCKDTSQTPLHCENLDTLAFILPHRTDNSESCVHGKHDSSWVEELLMLHRARITDVEHITGLSFYQQRKEPVSDILKLKTHLPTFSQED

SEQ ID NO: 16 - protein, 1155 aa, Artificial Sequence
  ENPP121 Fc
MERDGCAGGGSRGGEGGRAPREGPAGNGRDRGRSHAAEAPGDPQAAASLLAPMDVGEEPLEKAARARTAKDPNTYKIISLFTFAVGVNICLGFTAGLKPSCAKEVKSCKGRCFERTFGNCRCDAACVELGNCCLDYQETCIEPEHIWTCNKFRCGEKRLTRSLCACSDDCKDKGDCCINYSSVCQGEKSWVEEPCESINEPQCPAGFETPPTLLFSLDGFRAEYLHTWGGLLPVISKLKKCGTYTKNMRPVYPTKTFPNHYSIVTGLYPESHGIIDNKMYDPKMNASFSLKSKEKFNPEWYKGEPIWVTAKYQGLKSGTFFWPGSDVEINGIFPDIYKMYNGSVPFEERILAVLQWLQLPKDERPHFYTLYLEEPDSSGHSYGPVSSEVIKALQRVDGMVGMLMDGLKELNLHRCLNLILISDHGMEQGSCKKYIYLNKYLGDVKNIKVIYGPAARLRPSDVPDKYYSFNYEGIARNLSCREPNQHFKPYLKHFLPKRLHFAKSDRIEPLTFYLDPQWQLALNPSERKYCGSGFHGSDNVFSNMQALFVGYGPGFKHGIEADTFENIEVYNLMCDLLNLTPAPNNGTHGSLNHLLKNPVYTPKHPKEVHPLVQCPFTRNPRDNLGCSCNPSILPIEDFQTQFNLTVAEEKIIKHETLPYGRPRVLQKENTICLLSQHQFMSGYSQDILMPLWTSYTVDRNDSFSTEDFSNCLYQDFRIPLSPVHKCSFYKNNTKVSYGFLSPPQLNKNSSGIYSEALLTTNIVPMYQSFQVIWRYFHDTLLRKYAEERNGVNVVSGPVFDFDYDGRCDSLENLRQKRRVIRNQEILIPTHFFIVLTSCKDTSQTPLHCENLDTLAFILPHRTDNSESCVHGKHDSSWVEELLMLHRARITDVEHITGLSFYQQRKEPVSDILKLKTHLPTFSQEDLINDKTHTCPPCPAPELLGGPSVFLFPPKPKDTLMISRTPEVTCVVVDVSHEDPEVKFNWYVDGVEVHNAKTKPREEQYNSTYRVVSVLTVLHQDWLNGKEYKCKVSNKALPAPIEKTISKAKGQPREPQVYTLPPSREEMTKNQVSLTCLVKGFYPSDIAVEWESNGQPENNYKTTPPVLDSDGSFFLYSKLTVDKSRWQQGNVFSCSVMHEALHNHYTQKSLSLSPGK

SEQ ID NO: 17 - protein, 852 aa, Artificial Sequence
  ENNP71
MRGPAVLLTVALATLLAPGAGAGLKPSCAKEVKSCKGRCFERTFGNCRCDAACVELGNCCLDYQETCIEPEHIWTCNKFRCGEKRLTRSLCACSDDCKDKGDCCINYSSVCQGEKSWVEEPCESINEPQCPAGFETPPTLLFSLDGFRAEYLHTWGGLLPVISKLKKCGTYTKNMRPVYPTKTFPNHYSIVTGLYPESHGIIDNKMYDPKMNASFSLKSKEKFNPEWYKGEPIWVTAKYQGLKSGTFFWPGSDVEINGIFPDIYKMYNGSVPFEERILAVLQWLQLPKDERPHFYTLYLEEPDSSGHSYGPVSSEVIKALQRVDGMVGMLMDGLKELNLHRCLNLILISDHGMEQGSCKKYIYLNKYLGDVKNIKVIYGPAARLRPSDVPDKYYSFNYEGIARNLSCREPNQHFKPYLKHFLPKRLHFAKSDRIEPLTFYLDPQWQLALNPSERKYCGSGFHGSDNVFSNMQALFVGYGPGFKHGIEADTFENIEVYNLMCDLLNLTPAPNNGTHGSLNHLLKNPVYTPKHPKEVHPLVQCPFTRNPRDNLGCSCNPSILPIEDFQTQFNLTVAEEKIIKHETLPYGRPRVLQKENTICLLSQHQFMSGYSQDILMPLWTSYTVDRNDSFSTEDFSNCLYQDFRIPLSPVHKCSFYKNNTKVSYGFLSPPQLNKNSSGIYSEALLTTNIVPMYQSFQVIWRYFHDTLLRKYAEERNGVNVVSGPVFDFDYDGRCDSLENLRQKRRVIRNQEILIPTHFFIVLTSCKDTSQTPLHCENLDTLAFILPHRTDNSESCVHGKHDSSWVEELLMLHRARITDVEHITGLSFYQQRKEPVSDILKLKTHLPTFSQED

SEQ ID NO: 18 - protein, 1082 aa, Artificial Sequence
  ENPP71 Fc
MRGPAVLLTVALATLLAPGAGAGLKPSCAKEVKSCKGRCFERTFGNCRCDAACVELGNCCLDYQETCIEPEHIWTCNKFRCGEKRLTRSLCACSDDCKDKGDCCINYSSVCQGEKSWVEEPCESINEPQCPAGFETPPTLLFSLDGFRAEYLHTWGGLLPVISKLKKCGTYTKNMRPVYPTKTFPNHYSIVTGLYPESHGIIDNKMYDPKMNASFSLKSKEKFNPEWYKGEPIWVTAKYQGLKSGTFFWPGSDVEINGIFPDIYKMYNGSVPFEERILAVLQWLQLPKDERPHFYTLYLEEPDSSGHSYGPVSSEVIKALQRVDGMVGMLMDGLKELNLHRCLNLILISDHGMEQGSCKKYIYLNKYLGDVKNIKVIYGPAARLRPSDVPDKYYSFNYEGIARNLSCREPNQHFKPYLKHFLPKRLHFAKSDRIEPLTFYLDPQWQLALNPSERKYCGSGFHGSDNVFSNMQALFVGYGPGFKHGIEADTFENIEVYNLMCDLLNLTPAPNNGTHGSLNHLLKNPVYTPKHPKEVHPLVQCPFTRNPRDNLGCSCNPSILPIEDFQTQFNLTVAEEKIIKHETLPYGRPRVLQKENTICLLSQHQFMSGYSQDILMPLWTSYTVDRNDSFSTEDFSNCLYQDFRIPLSPVHKCSFYKNNTKVSYGFLSPPQLNKNSSGIYSEALLTTNIVPMYQSFQVIWRYFHDTLLRKYAEERNGVNVVSGPVFDFDYDGRCDSLENLRQKRRVIRNQEILIPTHFFIVLTSCKDTSQTPLHCENLDTLAFILPHRTDNSESCVHGKHDSSWVEELLMLHRARITDVEHITGLSFYQQRKEPVSDILKLKTHLPTFSQEDLINDKTHTCPPCPAPELLGGPSVFLFPPKPKDTLMISRTPEVTCVVVDVSHEDPEVKFNWYVDGVEVHNAKTKPREEQYNSTYRVVSVLTVLHQDWLNGKEYKCKVSNKALPAPIEKTISKAKGQPREPQVYTLPPSREEMTKNQVSLTCLVKGFYPSDIAVEWESNGQPENNYKTTPPVLDSDGSFFLYSKLTVDKSRWQQGNVFSCSVMHEALHNHYTQKSLSLSPGK

SEQ ID NO: 19 - protein, 849 aa, Artificial Sequence
  ENPP71 lacking ENPP1 N-Terminus GLK
MRGPAVLLTVALATLLAPGAGAPSCAKEVKSCKGRCFERTFGNCRCDAACVELGNCCLDYQETCIEPEHIWTCNKFRCGEKRLTRSLCACSDDCKDKGDCCINYSSVCQGEKSWVEEPCESINEPQCPAGFETPPTLLFSLDGFRAEYLHTWGGLLPVISKLKKCGTYTKNMRPVYPTKTFPNHYSIVTGLYPESHGIIDNKMYDPKMNASFSLKSKEKFNPEWYKGEPIWVTAKYQGLKSGTFFWPGSDVEINGIFPDIYKMYNGSVPFEERILAVLQWLQLPKDERPHFYTLYLEEPDSSGHSYGPVSSEVIKALQRVDGMVGMLMDGLKELNLHRCLNLILISDHGMEQGSCKKYIYLNKYLGDVKNIKVIYGPAARLRPSDVPDKYYSFNYEGIARNLSCREPNQHFKPYLKHFLPKRLHFAKSDRIEPLTFYLDPQWQLALNPSERKYCGSGFHGSDNVFSNMQALFVGYGPGFKHGIEADTFENIEVYNLMCDLLNLTPAPNNGTHGSLNHLLKNPVYTPKHPKEVHPLVQCPFTRNPRDNLGCSCNPSILPIEDFQTQFNLTVAEEKIIKHETLPYGRPRVLQKENTICLLSQHQFMSGYSQDILMPLWTSYTVDRNDSFSTEDFSNCLYQDFRIPLSPVHKCSFYKNNTKVSYGFLSPPQLNKNSSGIYSEALLTTNIVPMYQSFQVIWRYFHDTLLRKYAEERNGVNVVSGPVFDFDYDGRCDSLENLRQKRRVIRNQEILIPTHFFIVLTSCKDTSQTPLHCENLDTLAFILPHRTDNSESCVHGKHDSSWVEELLMLHRARITDVEHITGLSFYQQRKEPVSDILKLKTHLPTFSQED

SEQ ID NO: 20 - protein, 1079 aa, Artificial Sequence
  (ENPP71 lacking ENPP1 N-Terminus GLK)-Fc
MRGPAVLLTVALATLLAPGAGAPSCAKEVKSCKGRCFERTFGNCRCDAACVELGNCCLDYQETCIEPEHIWTCNKFRCGEKRLTRSLCACSDDCKDKGDCCINYSSVCQGEKSWVEEPCESINEPQCPAGFETPPTLLFSLDGFRAEYLHTWGGLLPVISKLKKCGTYTKNMRPVYPTKTFPNHYSIVTGLYPESHGIIDNKMYDPKMNASFSLKSKEKFNPEWYKGEPIWVTAKYQGLKSGTFFWPGSDVEINGIFPDIYKMYNGSVPFEERILAVLQWLQLPKDERPHFYTLYLEEPDSSGHSYGPVSSEVIKALQRVDGMVGMLMDGLKELNLHRCLNLILISDHGMEQGSCKKYIYLNKYLGDVKNIKVIYGPAARLRPSDVPDKYYSFNYEGIARNLSCREPNQHFKPYLKHFLPKRLHFAKSDRIEPLTFYLDPQWQLALNPSERKYCGSGFHGSDNVFSNMQALFVGYGPGFKHGIEADTFENIEVYNLMCDLLNLTPAPNNGTHGSLNHLLKNPVYTPKHPKEVHPLVQCPFTRNPRDNLGCSCNPSILPIEDFQTQFNLTVAEEKIIKHETLPYGRPRVLQKENTICLLSQHQFMSGYSQDILMPLWTSYTVDRNDSFSTEDFSNCLYQDFRIPLSPVHKCSFYKNNTKVSYGFLSPPQLNKNSSGIYSEALLTTNIVPMYQSFQVIWRYFHDTLLRKYAEERNGVNVVSGPVFDFDYDGRCDSLENLRQKRRVIRNQEILIPTHFFIVLTSCKDTSQTPLHCENLDTLAFILPHRTDNSESCVHGKHDSSWVEELLMLHRARITDVEHITGLSFYQQRKEPVSDILKLKTHLPTFSQEDLINDKTHTCPPCPAPELLGGPSVFLFPPKPKDTLMISRTPEVTCVVVDVSHEDPEVKFNWYVDGVEVHNAKTKPREEQYNSTYRVVSVLTVLHQDWLNGKEYKCKVSNKALPAPIEKTISKAKGQPREPQVYTLPPSREEMTKNQVSLTCLVKGFYPSDIAVEWESNGQPENNYKTTPPVLDSDGSFFLYSKLTVDKSRWQQGNVFSCSVMHEALHNHYTQKSLSLSPGK

SEQ ID NO: 21 - protein, 1550 aa, Artificial Sequence
  ENPP121-ALB
MERDGCAGGGSRGGEGGRAPREGPAGNGRDRGRSHAAEAPGDPQAAASLLAPMDVGEEPLEKAARARTAKDPNTYKIISLFTFAVGVNICLGFTAGLKPSCAKEVKSCKGRCFERTFGNCRCDAACVELGNCCLDYQETCIEPEHIWTCNKFRCGEKRLTRSLCACSDDCKDKGDCCINYSSVCQGEKSWVEEPCESINEPQCPAGFETPPTLLFSLDGFRAEYLHTWGGLLPVISKLKKCGTYTKNMRPVYPTKTFPNHYSIVTGLYPESHGIIDNKMYDPKMNASFSLKSKEKFNPEWYKGEPIWVTAKYQGLKSGTFFWPGSDVEINGIFPDIYKMYNGSVPFEERILAVLQWLQLPKDERPHFYTLYLEEPDSSGHSYGPVSSEVIKALQRVDGMVGMLMDGLKELNLHRCLNLILISDHGMEQGSCKKYIYLNKYLGDVKNIKVIYGPAARLRPSDVPDKYYSFNYEGIARNLSCREPNQHFKPYLKHFLPKRLHFAKSDRIEPLTFYLDPQWQLALNPSERKYCGSGFHGSDNVFSNMQALFVGYGPGFKHGIEADTFENIEVYNLMCDLLNLTPAPNNGTHGSLNHLLKNPVYTPKHPKEVHPLVQCPFTRNPRDNLGCSCNPSILPIEDFQTQFNLTVAEEKIIKHETLPYGRPRVLQKENTICLLSQHQFMSGYSQDILMPLWTSYTVDRNDSFSTEDFSNCLYQDFRIPLSPVHKCSFYKNNTKVSYGFLSPPQLNKNSSGIYSEALLTTNIVPMYQSFQVIWRYFHDTLLRKYAEERNGVNVVSGPVFDFDYDGRCDSLENLRQKRRVIRNQEILIPTHFFIVLTSCKDTSQTPLHCENLDTLAFILPHRTDNSESCVHGKHDSSWVEELLMLHRARITDVEHITGLSFYQQRKEPVSDILKLKTHLPTFSQEDRSGSGGSMKWVTFLLLLFVSGSAFSRGVFRREAHKSEIAHRYNDLGEQHFKGLVLIAFSQYLQKCSYDEHAKLVQEVTDFAKTCVADESAANCDKSLHTLFGDKLCAIPNLRENYGELADCCTKQEPERNECFLQHKDDNPSLPPFERPEAEAMCTSFKENPTTFMGHYLHEVARRHPYFYAPELLYYAEQYNEILTQCCAEADKESCLTPKLDGVKEKALVSSVRQRMKCSSMQKFGERAFKAWAVARLSQTFPNADFAEITKLATDLTKVNKECCHGDLLECADDRAELAKYMCENQATISSKLQTCCDKPLLKKAHCLSEVEHDTMPADLPAIAADFVEDQEVCKNYAEAKDVFLGTFLYEYSRRHPDYSVSLLLRLAKKYEATLEKCCAEANPPACYGTVLAEFQPLVEEPKNLVKTNCDLYEKLGEYGFQNAILVRYTQKAPQVSTPTLVEAARNLGRVGTKCCTLPEDQRLPCVEDYLSAILNRVCLLHEKTPVSEHVTKCCSGSLVERRPCFSALTVDETYVPKEFKAETFTFHSDICTLPEKEKQIKKQTALAELVKHKPKATAEQLKTVMDDFAQFLDTCCKAADKDTCFSTEGPNLVTRCKDALARSWSHPQFEK

SEQ ID NO: 22 - protein, 1474 aa, Artificial Sequence
  (ENPP71 lacking ENPP1 N-Terminus GLK)-ALB
MRGPAVLLTVALATLLAPGAGAPSCAKEVKSCKGRCFERTFGNCRCDAACVELGNCCLDYQETCIEPEHIWTCNKFRCGEKRLTRSLCACSDDCKDKGDCCINYSSVCQGEKSWVEEPCESINEPQCPAGFETPPTLLFSLDGFRAEYLHTWGGLLPVISKLKKCGTYTKNMRPVYPTKTFPNHYSIVTGLYPESHGIIDNKMYDPKMNASFSLKSKEKFNPEWYKGEPIWVTAKYQGLKSGTFFWPGSDVEINGIFPDIYKMYNGSVPFEERILAVLQWLQLPKDERPHFYTLYLEEPDSSGHSYGPVSSEVIKALQRVDGMVGMLMDGLKELNLHRCLNLILISDHGMEQGSCKKYIYLNKYLGDVKNIKVIYGPAARLRPSDVPDKYYSFNYEGIARNLSCREPNQHFKPYLKHFLPKRLHFAKSDRIEPLTFYLDPQWQLALNPSERKYCGSGFHGSDNVFSNMQALFVGYGPGFKHGIEADTFENIEVYNLMCDLLNLTPAPNNGTHGSLNHLLKNPVYTPKHPKEVHPLVQCPFTRNPRDNLGCSCNPSILPIEDFQTQFNLTVAEEKIIKHETLPYGRPRVLQKENTICLLSQHQFMSGYSQDILMPLWTSYTVDRNDSFSTEDFSNCLYQDFRIPLSPVHKCSFYKNNTKVSYGFLSPPQLNKNSSGIYSEALLTTNIVPMYQSFQVIWRYFHDTLLRKYAEERNGVNVVSGPVFDFDYDGRCDSLENLRQKRRVIRNQEILIPTHFFIVLTSCKDTSQTPLHCENLDTLAFILPHRTDNSESCVHGKHDSSWVEELLMLHRARITDVEHITGLSFYQQRKEPVSDILKLKTHLPTFSQEDRSGSGGSMKWVTFLLLLFVSGSAFSRGVFRREAHKSEIAHRYNDLGEQHFKGLVLIAFSQYLQKCSYDEHAKLVQEVTDFAKTCVADESAANCDKSLHTLFGDKLCAIPNLRENYGELADCCTKQEPERNECFLQHKDDNPSLPPFERPEAEAMCTSFKENPTTFMGHYLHEVARRHPYFYAPELLYYAEQYNEILTQCCAEADKESCLTPKLDGVKEKALVSSVRQRMKCSSMQKFGERAFKAWAVARLSQTFPNADFAEITKLATDLTKVNKECCHGDLLECADDRAELAKYMCENQATISSKLQTCCDKPLLKKAHCLSEVEHDTMPADLPAIAADFVEDQEVCKNYAEAKDVFLGTFLYEYSRRHPDYSVSLLLRLAKKYEATLEKCCAEANPPACYGTVLAEFQPLVEEPKNLVKTNCDLYEKLGEYGFQNAILVRYTQKAPQVSTPTLVEAARNLGRVGTKCCTLPEDQRLPCVEDYLSAILNRVCLLHEKTPVSEHVTKCCSGSLVERRPCFSALTVDETYVPKEFKAETFTFHSDICTLPEKEKQIKKQTALAELVKHKPKATAEQLKTVMDDFAQFLDTCCKAADKDTCFSTEGPNLVTRCKDALARSWSHPQFEK

SEQ ID NO: 23 - protein, 19 aa, Artificial Sequence
  chemically synthesized
IISLFTFAVGVNICLGFTA

SEQ ID NO: 24 - protein, 850 aa, Artificial Sequence
  ENPP51
MTSKFLLVSFILAALSLSTTFSLQPSCAKEVKSCKGRCFERTFSNCRCDAACVSLGNCCLDFQETCVEPTHIWTCNKFRCGEKRLSRFVCSCADDCKTHNDCCINYSSVCQDKKSWVEETCESIDTPECPAEFESPPTLLFSLDGFRAEYLHTWGGLLPVISKLKNCGTYTKNMRPMYPTKTFPNHYSIVTGLYPESHGIIDNKMYDPKMNASFSLKSKEKFNPLWYKGQPIWVTANHQEVKSGTYFWPGSDVEIDGILPDIYKVYNGSVPFEERILAVLEWLQLPSHERPHFYTLYLEEPDSSGHSHGPVSSEVIKALQKVDRLVGMLMDGLKDLGLDKCLNLILISDHGMEQGSCKKYVYLNKYLGDVNNVKVVYGPAARLRPTDVPETYYSFNYEALAKNLSCREPNQHFRPYLKPFLPKRLHFAKSDRIEPLTFYLDPQWQLALNPSERKYCGSGFHGSDNLFSNMQALFIGYGPAFKHGAEVDSFENIEVYNLMCDLLGLIPAPNNGSHGSLNHLLKKPIYNPSHPKEEGFLSQCPIKSTSNDLGCTCDPWIVPIKDFEKQLNLTTEDVDDIYHMTVPYGRPRILLKQHRVCLLQQQQFLTGYSLDLLMPLWASYTFLSNDQFSRDDFSNCLYQDLRIPLSPVHKCSYYKSNSKLSYGFLTPPRLNRVSNHIYSEALLTSNIVPMYQSFQVIWHYLHDTLLQRYAHERNGINVVSGPVFDFDYDGRYDSLEILKQNSRVIRSQEILIPTHFFIVLTSCKQLSETPLECSALESSAYILPHRPDNIESCTHGKRESSWVEELLTLHRARVTDVELITGLSFYQDRQESVSELLRLKTHLPIFSQED

SEQ ID NO: 25 - protein, 1474 aa, Artificial Sequence
  ENPP51-ALB
MTSKFLLVSFILAALSLSTTFSLQPSCAKEVKSCKGRCFERTFSNCRCDAACVSLGNCCLDFQETCVEPTHIWTCNKFRCGEKRLSRFVCSCADDCKTHNDCCINYSSVCQDKKSWVEETCESIDTPECPAEFESPPTLLFSLDGFRAEYLHTWGGLLPVISKLKNCGTYTKNMRPMYPTKTFPNHYSIVTGLYPESHGIIDNKMYDPKMNASFSLKSKEKFNPLWYKGQPIWVTANHQEVKSGTYFWPGSDVEIDGILPDIYKVYNGSVPFEERILAVLEWLQLPSHERPHFYTLYLEEPDSSGHSHGPVSSEVIKALQKVDRLVGMLMDGLKDLGLDKCLNLILISDHGMEQGSCKKYVYLNKYLGDVNNVKVVYGPAARLRPTDVPETYYSFNYEALAKNLSCREPNQHFRPYLKPFLPKRLHFAKSDRIEPLTFYLDPQWQLALNPSERKYCGSGFHGSDNLFSNMQALFIGYGPAFKHGAEVDSFENIEVYNLMCDLLGLIPAPNNGSHGSLNHLLKKPIYNPSHPKEEGFLSQCPIKSTSNDLGCTCDPWIVPIKDFEKQLNLTTEDVDDIYHMTVPYGRPRILLKQHRVCLLQQQQFLTGYSLDLLMPLWASYTFLSNDQFSRDDFSNCLYQDLRIPLSPVHKCSYYKSNSKLSYGFLTPPRLNRVSNHIYSEALLTSNIVPMYQSFQVIWHYLHDTLLQRYAHERNGINVVSGPVFDFDYDGRYDSLEILKQNSRVIRSQEILIPTHFFIVLTSCKQLSETPLECSALESSAYILPHRPDNIESCTHGKRESSWVEELLTLHRARVTDVELITGLSFYQDRQESVSELLRLKTHLPIFSQEDGGSGGSMKWVTFLLLLFVSGSAFSRGVFRREAHKSEIAHRYNDLGEQHFKGLVLIAFSQYLQKCSYDEHAKLVQEVTDFAKTCVADESAANCDKSLHTLFGDKLCAIPNLRENYGELADCCTKQEPERNECFLQHKDDNPSLPPFERPEAEAMCTSFKENPTTFMGHYLHEVARRHPYFYAPELLYYAEQYNEILTQCCAEADKESCLTPKLDGVKEKALVSSVRQRMKCSSMQKFGERAFKAWAVARLSQTFPNADFAEITKLATDLTKVNKECCHGDLLECADDRAELAKYMCENQATISSKLQTCCDKPLLKKAHCLSEVEHDTMPADLPAIAADFVEDQEVCKNYAEAKDVFLGTFLYEYSRRHPDYSVSLLLRLAKKYEATLEKCCAEANPPACYGTVLAEFQPLVEEPKNLVKTNCDLYEKLGEYGFQNAILVRYTQKAPQVSTPTLVEAARNLGRVGTKCCTLPEDQRLPCVEDYLSAILNRVCLLHEKTPVSEHVTKCCSGSLVERRPCFSALTVDETYVPKEFKAETFTFHSDICTLPEKEKQIKKQTALAELVKHKPKATAEQLKTVMDDFAQFLDTCCKAADKDTCFSTEGPNLVTRCKDALARSWSHPQFEK

SEQ ID NO: 26 - protein, 227 aa, Artificial Sequence
  Human IgG Fc domain, Fc
DKTHTCPPCPAPELLGGPSVFLFPPKPKDTLMISRTPEVTCVVVDVSHEDPEVKFNWYVDGVEVHNAKTKPREEQYNSTYRVVSVLTVLHQDWLNGKEYKCKVSNKALPAPIEKTISKAKGQPREPQVYTLPPSREEMTKNQVSLTCLVKGFYPSDIAVEWESNGQPENNYKTTPPVLDSDGSFFLYSKLTVDKSRWQQGNVFSCSVMHEALHNHYTQKSLSLSPGK

SEQ ID NO: 27 - protein, 618 aa, Artificial Sequence
  ALB
MKWVTFLLLLFVSGSAFSRGVFRREAHKSEIAHRYNDLGEQHFKGLVLIAFSQYLQKCSYDEHAKLVQEVTDFAKTCVADESAANCDKSLHTLFGDKLCAIPNLRENYGELADCCTKQEPERNECFLQHKDDNPSLPPFERPEAEAMCTSFKENPTTFMGHYLHEVARRHPYFYAPELLYYAEQYNEILTQCCAEADKESCLTPKLDGVKEKALVSSVRQRMKCSSMQKFGERAFKAWAVARLSQTFPNADFAEITKLATDLTKVNKECCHGDLLECADDRAELAKYMCENQATISSKLQTCCDKPLLKKAHCLSEVEHDTMPADLPAIAADFVEDQEVCKNYAEAKDVFLGTFLYEYSRRHPDYSVSLLLRLAKKYEATLEKCCAEANPPACYGTVLAEFQPLVEEPKNLVKTNCDLYEKLGEYGFQNAILVRYTQKAPQVSTPTLVEAARNLGRVGTKCCTLPEDQRLPCVEDYLSAILNRVCLLHEKTPVSEHVTKCCSGSLVERRPCFSALTVDETYVPKEFKAETFTFHSDICTLPEKEKQIKKQTALAELVKHKPKATAEQLKTVMDDFAQFLDTCCKAADKDTCFSTEGPNLVTRCKDALARSWSHPQFEK

SEQ ID NO: 28 - protein, 3 aa, Artificial Sequence
  chemically synthesized
LIN

SEQ ID NO: 29 - protein, 6 aa, Artificial Sequence
  chemically synthesized
GGSGGS

SEQ ID NO: 30 - protein, 7 aa, Artificial Sequence
  chemically synthesized
RSGSGGS

SEQ ID NO: 31 - protein, 875 aa, Homo sapiens [sequence omitted]

SEQ ID NO: 32 - protein, 827 aa, Artificial Sequence
  Extracellular domain of ENPP3
EKQGSCRKKCFDASFRGLENCRCDVACKDRGDCCWDFEDTCVESTRIWMCNKFRCGETRLEASLCSCSDDCLQRKDCCADYKSVCQGETSWLEENCDTAQQSQCPEGFDLPPVILFSMDGFRAEYLYTWDTLMPNINKLKTCGIHSKYMRAMYPTKTFPNHYTIVTGLYPESHGIIDNNMYDVNLNKNFSLSSKEQNNPAWWHGQPMWLTAMYQGLKAATYFWPGSEVAINGSFPSIYMPYNGSVPFEERISTLLKWLDLPKAERPRFYTMYFEEPDSSGHAGGPVSARVIKALQVVDHAFGMLMEGLKQRNLHNCVNIILLADHGMDQTYCNKMEYMTDYFPRINFFYMYEGPAPRIRAHNIPHDFFSFNSEEIVRNLSCRKPDQHFKPYLTPDLPKRLHYAKNVRIDKVHLFVDQQWLAVRSKSNTNCGGGNHGYNNEFRSMEAIFLAHGPSFKEKTEVEPFENIEVYNLMCDLLRIQPAPNNGTHGSLNHLLKVPFYEPSHAEEVSKFSVCGFANPLPTESLDCFCPHLQNSTQLEQVNQMLNLTQEEITATVKVNLPFGRPRVLQKNVDHCLLYHREYVSGFGKAMRMPMWSSYTVPQLGDTSPLPPTVPDCLRADVRVPPSESQKCSFYLADKNITHGFLYPPASNRTSDSQYDALITSNLVPMYEEFRKMWDYFHSVLLIKHATERNGVNVVSGPIFDYNYDGHFDAPDEITKHLANTDVPIPTHYFVVLTSCKNKSHTPENCPGWLDVLPFIIPHRPTNVESCPEGKPEALWVEERFTAHIARVRDVELLTGLDFYQDKVQPVSEILQLKTYLPTFETTI

SEQ ID NO: 33 - protein, 17 aa, Artificial Sequence
  exENPP3
LLVIMSLGLGLGLGLRK

SEQ ID NO: 34 - protein, 22 aa, Artificial Sequence
  ENPP7 protein export signal sequence
MRGPAVLLTVALATLLAPGAGA

SEQ ID NO: 35 - protein, 98 aa, Artificial Sequence
  ENPP121GLK protein export signal sequence
MERDGCAGGGSRGGEGGRAPREGPAGNGRDRGRSHAAEAPGDPQAAASLLAPMDVGEEPLEKAARARTAKDPNTYKIISLFTFAVGVNICLGFTAGLK

SEQ ID NO: 36 - protein, 95 aa, Artificial Sequence
  ENPP121 protein export signal sequence
MERDGCAGGGSRGGEGGRAPREGPAGNGRDRGRSHAAEAPGDPQAAASLLAPMDVGEEPLEKAARARTAKDPNTYKIISLFTFAVGVNICLGFTA

SEQ ID NO: 37 - protein, 23 aa, Artificial Sequence
  ENPP5 protein export signal sequence
  MOD_RES (23)..(23): residue can be absent, L, or LQ
MTSKFLLVSFILAALSLSTTFSX

SEQ ID NO: 38 - protein, 20 aa, Artificial Sequence
  ENPP7 signal sequence
MRGPAVLLTVALATLLAPGA

SEQ ID NO: 39 - protein, 22 aa, Artificial Sequence
  ENPP7 signal sequence
MRGPAVLLTVALATLLAPGAGA

SEQ ID NO: 40 - protein, 16 aa, Artificial Sequence
  chemically synthesized
LVIMSLGLGLGLGLRK

SEQ ID NO: 41 - protein, 15 aa, Artificial Sequence
  chemically synthesized
VIMSLGLGLGLGLRK

SEQ ID NO: 42 - protein, 14 aa, Artificial Sequence
  chemically synthesized
IMSLGLGLGLGLRK

SEQ ID NO: 43 - protein, 13 aa, Artificial Sequence
  chemically synthesized
MSLGLGLGLGLRK

SEQ ID NO: 44 - protein, 12 aa, Artificial Sequence
  chemically synthesized
SLGLGLGLGLRK

SEQ ID NO: 45 - protein, 11 aa, Artificial Sequence
  chemically synthesized
LGLGLGLGLRK

SEQ ID NO: 46 - protein, 10 aa, Artificial Sequence
  chemically synthesized
GLGLGLGLRK

SEQ ID NO: 47 - protein, 9 aa, Artificial Sequence
  chemically synthesized
LGLGLGLRK

SEQ ID NO: 48 - protein, 8 aa, Artificial Sequence
  chemically synthesized
GLGLGLRK

SEQ ID NO: 49 - protein, 7 aa, Artificial Sequence
  chemically synthesized
LGLGLRK

SEQ ID NO: 50 - protein, 6 aa, Artificial Sequence
  chemically synthesized
GLGLRK

SEQ ID NO: 51 - protein, 5 aa, Artificial Sequence
  chemically synthesized
LGLRK

SEQ ID NO: 52 - protein, 4 aa, Artificial Sequence
  chemically synthesized
GLRK

SEQ ID NO: 53 - protein, 3 aa, Artificial Sequence
  chemically synthesized
LRK

SEQ ID NO: 54 - protein, 2 aa, Artificial Sequence
  chemically synthesized
RK

SEQ ID NO: 55 - protein, 1 aa, Artificial Sequence
  chemically synthesized
K

SEQ ID NO: 56 - protein, 1147 aa, Artificial Sequence
  ENPP121-NPP3-Fc
MERDGCAGGGSRGGEGGRAPREGPAGNGRDRGRSHAAEAPGDPQAAASLLAPMDVGEEPLEKAARARTAKDPNTYKIISLFTFAVGVNICLGFTAKQGSCRKKCFDASFRGLENCRCDVACKDRGDCCWDFEDTCVESTRIWMCNKFRCGERLEASLCSCSDDCLQRKDCCADYKSVCQGETSWLEENCDTAQQSQCPEGFDLPPVILFSMDGFRAEYLYTWDTLMPNINKLKTCGIHSKYMRAMYPTKTFPNHYTIVTGLYPESHGIIDNNMYDVNLNKNFSLSSKEQNNPAWWHGQPMWLTAMYQGLKAATYFWPGSEVAINGSFPSIYMPYNGSVPFEERISTLLKWLDLPKAERPRFYTMYFEEPDSSGHAGGPVSARVIKALQVVDHAFGMLMEGLKQRNLHNCVNIILLADHGMDQTYCNKMEYMTDYFPRINFFYMYEGPAPRIRAHNIPHDFFSFNSEEIVRNLSCRKPDQHFKPYLTPDLPKRLHYAKNVRIDKVHLFVDQQWLAVRSKSNTNCGGGNHGYNNEFRSMEAIFLAHGPSFKEKTEVEPFENIEVYNLMCDLLRIQPAPNNGTHGSLNHLLKVPFYEPSHAEEVSKFSVCGFANPLPTESLDCFCPHLQNSTQLEQVNQMLNLTQEEITATVKVNLPFGRPRVLQKNVDHCLLYHREYVSGFGKAMRMPMWSSYTVPQLGDTSPLPPTVPDCLRADVRVPPSESQKCSFYLADKNITHGFLYPPASNRTSDSQYDALITSNLVPMYEEFRKMWDYFHSVLLIKHATERNGVNVVSGPIFDYNYDGHFDAPDEITKHLANTDVPIPTHYFVVLTSCKNKSHTPENCPGWLDVLPFIIPHRPTNVESCPEGKPEALWVEERFTAHIARVRDVELLTGLDFYQDKVQPVSEILQLKTYLPTFETTIDKTHTCPPCPAPELLGGPSVFLFPPKPKDTLMISRTPEVTCVVVDVSHEDPEVKFNWYVDGVEVHNAKTKPREEQYNSTYRVVSVLTVLHQDWLNGKEYKCKVSNKALPAPIEKTISKAKGQPREPQVYTLPPSREEMTKNQVSLTCLVKGFYPSDIAVEWESNGQPENNYKTTPPVLDSDGSFFLYSKLTVDKSRWQQGNVFSCSVMHEALHNHYTQKSLSLSPGK

SEQ ID NO: 57 - protein, 1072 aa, Artificial Sequence
  ENPP7-ENPP3-Fc
MRGPAVLLTVALATLLAPGAKQGSCRKKCFDASFRGLENCRCDVACKDRGDCCWDFEDTCVESTRIWMCNKFRCGERLEASLCSCSDDCLQRKDCCADYKSVCQGETSWLEENCDTAQQSQCPEGFDLPPVILFSMDGFRAEYLYTWDTLMPNINKLKTCGIHSKYMRAMYPTKTFPNHYTIVTGLYPESHGIIDNNMYDVNLNKNFSLSSKEQNNPAWWHGQPMWLTAMYQGLKAATYFWPGSEVAINGSFPSIYMPYNGSVPFEERISTLLKWLDLPKAERPRFYTMYFEEPDSSGHAGGPVSARVIKALQVVDHAFGMLMEGLKQRNLHNCVNIILLADHGMDQTYCNKMEYMTDYFPRINFFYMYEGPAPRIRAHNIPHDFFSFNSEEIVRNLSCRKPDQHFKPYLTPDLPKRLHYAKNVRIDKVHLFVDQQWLAVRSKSNTNCGGGNHGYNNEFRSMEAIFLAHGPSFKEKTEVEPFENIEVYNLMCDLLRIQPAPNNGTHGSLNHLLKVPFYEPSHAEEVSKFSVCGFANPLPTESLDCFCPHLQNSTQLEQVNQMLNLTQEEITATVKVNLPFGRPRVLQKNVDHCLLYHREYVSGFGKAMRMPMWSSYTVPQLGDTSPLPPTVPDCLRADVRVPPSESQKCSFYLADKNITHGFLYPPASNRTSDSQYDALITSNLVPMYEEFRKMWDYFHSVLLIKHATERNGVNVVSGPIFDYNYDGHFDAPDEITKHLANTDVPIPTHYFVVLTSCKNKSHTPENCPGWLDVLPFIIPHRPTNVESCPEGKPEALWVEERFTAHIARVRDVELLTGLDFYQDKVQPVSEILQLKTYLPTFETTIDKTHTCPPCPAPELLGGPSVFLFPPKPKDTLMISRTPEVTCVVVDVSHEDPEVKFNWYVDGVEVHNAKTKPREEQYNSTYRVVSVLTVLHQDWLNGKEYKCKVSNKALPAPIEKTISKAKGQPREPQVYTLPPSREEMTKNQVSLTCLVKGFYPSDIAVEWESNGQPENNYKTTPPVLDSDGSFFLYSKLTVDKSRWQQGNVFSCSVMHEALHNHYTQKSLSLSPGK

SEQ ID NO: 58 - protein, 1074 aa, Artificial Sequence
  ENPP5-ENPP3-Fc
MTSKFLLVSFILAALSLSTTFSKQGSCRKKCFDASFRGLENCRCDVACKDRGDCCWDFEDTCVESTRIWMCNKFRCGERLEASLCSCSDDCLQRKDCCADYKSVCQGETSWLEENCDTAQQSQCPEGFDLPPVILFSMDGFRAEYLYTWDTLMPNINKLKTCGIHSKYMRAMYPTKTFPNHYTIVTGLYPESHGIIDNNMYDVNLNKNFSLSSKEQNNPAWWHGQPMWLTAMYQGLKAATYFWPGSEVAINGSFPSIYMPYNGSVPFEERISTLLKWLDLPKAERPRFYTMYFEEPDSSGHAGGPVSARVIKALQVVDHAFGMLMEGLKQRNLHNCVNIILLADHGMDQTYCNKMEYMTDYFPRINFFYMYEGPAPRIRAHNIPHDFFSFNSEEIVRNLSCRKPDQHFKPYLTPDLPKRLHYAKNVRIDKVHLFVDQQWLAVRSKSNTNCGGGNHGYNNEFRSMEAIFLAHGPSFKEKTEVEPFENIEVYNLMCDLLRIQPAPNNGTHGSLNHLLKVPFYEPSHAEEVSKFSVCGFANPLPTESLDCFCPHLQNSTQLEQVNQMLNLTQEEITATVKVNLPFGRPRVLQKNVDHCLLYHREYVSGFGKAMRMPMWSSYTVPQLGDTSPLPPTVPDCLRADVRVPPSESQKCSFYLADKNITHGFLYPPASNRTSDSQYDALITSNLVPMYEEFRKMWDYFHSVLLIKHATERNGVNVVSGPIFDYNYDGHFDAPDEITKHLANTDVPIPTHYFVVLTSCKNKSHTPENCPGWLDVLPFIIPHRPTNVESCPEGKPEALWVEERFTAHIARVRDVELLTGLDFYQDKVQPVSEILQLKTYLPTFETTIDKTHTCPPCPAPELLGGPSVFLFPPKPKDTLMISRTPEVTCVVVDVSHEDPEVKFNWYVDGVEVHNAKTKPREEQYNSTYRVVSVLTVLHQDWLNGKEYKCKVSNKALPAPIEKTISKAKGQPREPQVYTLPPSREEMTKNQVSLTCLVKGFYPSDIAVEWESNGQPENNYKTTPPVLDSDGSFFLYSKLTVDKSRWQQGNVFSCSVMHEALHNHYTQKSLSLSPGK

SEQ ID NO: 59 - protein, 623 aa, Homo sapiens
GGGGSGGGGSGGGGSMKWVTFLLLLFVSGSAFSRGVFRREAHKSEIAHRYNDLGEQHFKGLVLIAFSQYLQKCSYDEHAKLVQEVTDFAKTCVADESAANCDKSLHTLFGDKLCAIPNLRENYGELADCCTKQEPERNECFLQHKDDNPSLPPFERPEAEAMCTSFKENPTTFMGHYLHEVARRHPYFYAPELLYYAEQYNEILTQCCAEADKESCLTPKLDGVKEKALVSSVRQRMKCSSMQKFGERAFKAWAVARLSQTFPNADFAEITKLATDLTKVNKECCHGDLLECADDRAELAKYMCENQATISSKLQTCCDKPLLKKAHCLSEVEHDTMPADLPAIAADFVEDQEVCKNYAEAKDVFLGTFLYEYSRRHPDYSVSLLLRLAKKYEATLEKCCAEANPPACYGTVLAEFQPLVEEPKNLVKTNCDLYEKLGEYGFQNAILVRYTQKAPQVSTPTLVEAARNLGRVGTKCCTLPEDQRLPCVEDYLSAILNRVCLLHEKTPVSEHVTKCCSGSLVERRPCFSALTVDETYVPKEFKAETFTFHSDICTLPEKEKQIKKQTALAELVKHKPKATAEQLKTVMDDFAQFLDTCCKAADKDTCFSTEGPNLVTRCKDALA

SEQ ID NO: 60 - protein, 1582 aa, Artificial Sequence
  ENPP121-ENPP3-Albumin
MERDGCAGGGSRGGEGGRAPREGPAGNGRDRGRSHAAEAPGDPQAAASLLAPMDVGEEPLEKAARARTAKDPNTYKIISLFTFAVGVNICLGFTAKQGSCRKKCFDASFRGLENCRCDVACKDRGDCCWDFEDTCVESTRIWMCNKFRCGERLEASLCSCSDDCLQRKDCCADYKSVCQGETSWLEENCDTAQQSQCPEGFDLPPVILFSMDGFRAEYLYTWDTLMPNINKLKTCGIHSKYMRAMYPTKTFPNHYTIVTGLYPESHGIIDNNMYDVNLNKNFSLSSKEQNNPAWWHGQPMWLTAMYQGLKAATYFWPGSEVAINGSFPSIYMPYNGSVPFEERISTLLKWLDLPKAERPRFYTMYFEEPDSSGHAGGPVSARVIKALQVVDHAFGMLMEGLKQRNLHNCVNIILLADHGMDQTYCNKMEYMTDYFPRINFFYMYEGPAPRIRAHNIPHDFFSFNSEEIVRNLSCRKPDQHFKPYLTPDLPKRLHYAKNVRIDKVHLFVDQQWLAVRSKSNTNCGGGNHGYNNEFRSMEAIFLAHGPSFKEKTEVEPFENIEVYNLMCDLLRIQPAPNNGTHGSLNHLLKVPFYEPSHAEEVSKFSVCGFANPLPTESLDCFCPHLQNSTQLEQVNQMLNLTQEEITATVKVNLPFGRPRVLQKNVDHCLLYHREYVSGFGKAMRMPMWSSYTVPQLGDTSPLPPTVPDCLRADVRVPPSESQKCSFYLADKNITHGFLYPPASNRTSDSQYDALITSNLVPMYEEFRKMWDYFHSVLLIKHATERNGVNVVSGPIFDYNYDGHFDAPDEITKHLANTDVPIPTHYFVVLTSCKNKSHTPENCPGWLDVLPFIIPHRPTNVESCPEGKPEALWVEERFTAHIARVRDVELLTGLDFYQDKVQPVSEILQLKTYLPTFETTIDKTHTCPPCPAPELLGGPSVFLFPPKPKDTLMISRTPEVTGGGSGGGGSGGGGSMKWVTFLLLLFVSGSAFSRGVFRREAHKSEIAHRYNDLGEQHFKGLVLIAFSQYLQKCSYDEHAKLVQEVTDFAKTCVADESAANCDKSLHTLFGDKLCAIPNLRENYGELADCCTKQEPERNECFLQHKDDNPSLPPFERPEAEAMCTSFKENPTTFMGHYLHEVARRHPYFYAPELLYYAEQYNEILTQCCAEADKESCLTPKLDGVKEKALVSSVRQRMKCSSMQKFGERAFKAWAVARLSQTFPNADFAEITKLATDLTKVNKECCHGDLLECADDRAELAKYMCENQATISSKLQTCCDKPLLKKAHCLSEVEHDTMPADLPAIAADFVEDQEVCKNYAEAKDVFLGTFLYEYSRRHPDYSVSLLLRLAKKYEATLEKCCAEANPPACYGTVLAEFQPLVEEPKNLVKTNCDLYEKLGEYGFQNAILVRYTQKAPQVSTPTLVEAARNLGRVGTKCCTLPEDQRLPCVEDYLSAILNRVCLLHEKTPVSEHVTKCCSGSLVERRPCFSALTVDETYVPKEFKAETFTFHSDICTLPEKEKQIKKQTALAELVKHKPKATAEQLKTVMDDFAQFLDTCCKAADKDTCFSTEGPNLVTRCKDALA

SEQ ID NO: 61 - protein, 1507 aa, Artificial Sequence
  ENPP7-ENPP3-Albumin
MRGPAVLLTVALATLLAPGAKQGSCRKKCFDASFRGLENCRCDVACKDRGDCCWDFEDTCVESTRIWMCNKFRCGERLEASLCSCSDDCLQRKDCCADYKSVCQGETSWLEENCDTAQQSQCPEGFDLPPVILFSMDGFRAEYLYTWDTLMPNINKLKTCGIHSKYMRAMYPTKTFPNHYTIVTGLYPESHGIIDNNMYDVNLNKNFSLSSKEQNNPAWWHGQPMWLTAMYQGLKAATYFWPGSEVAINGSFPSIYMPYNGSVPFEERISTLLKWLDLPKAERPRFYTMYFEEPDSSGHAGGPVSARVIKALQVVDHAFGMLMEGLKQRNLHNCVNIILLADHGMDQTYCNKMEYMTDYFPRINFFYMYEGPAPRIRAHNIPHDFFSFNSEEIVRNLSCRKPDQHFKPYLTPDLPKRLHYAKNVRIDKVHLFVDQQWLAVRSKSNTNCGGGNHGYNNEFRSMEAIFLAHGPSFKEKTEVEPFENIEVYNLMCDLLRIQPAPNNGTHGSLNHLLKVPFYEPSHAEEVSKFSVCGFANPLPTESLDCFCPHLQNSTQLEQVNQMLNLTQEEITATVKVNLPFGRPRVLQKNVDHCLLYHREYVSGFGKAMRMPMWSSYTVPQLGDTSPLPPTVPDCLRADVRVPPSESQKCSFYLADKNITHGFLYPPASNRTSDSQYDALITSNLVPMYEEFRKMWDYFHSVLLIKHATERNGVNVVSGPIFDYNYDGHFDAPDEITKHLANTDVPIPTHYFVVLTSCKNKSHTPENCPGWLDVLPFIIPHRPTNVESCPEGKPEALWVEERFTAHIARVRDVELLTGLDFYQDKVQPVSEILQLKTYLPTFETTIDKTHTCPPCPAPELLGGPSVFLFPPKPKDTLMISRTPEVTGGGSGGGGSGGGGSMKWVTFLLLLFVSGSAFSRGVFRREAHKSEIAHRYNDLGEQHFKGLVLIAFSQYLQKCSYDEHAKLVQEVTDFAKTCVADESAANCDKSLHTLFGDKLCAIPNLRENYGELADCCTKQEPERNECFLQHKDDNPSLPPFERPEAEAMCTSFKENPTTFMGHYLHEVARRHPYFYAPELLYYAEQYNEILTQCCAEADKESCLTPKLDGVKEKALVSSVRQRMKCSSMQKFGERAFKAWAVARLSQTFPNADFAEITKLATDLTKVNKECCHGDLLECADDRAELAKYMCENQATISSKLQTCCDKPLLKKAHCLSEVEHDTMPADLPAIAADFVEDQEVCKNYAEAKDVFLGTFLYEYSRRHPDYSVSLLLRLAKKYEATLEKCCAEANPPACYGTVLAEFQPLVEEPKNLVKTNCDLYEKLGEYGFQNAILVRYTQKAPQVSTPTLVEAARNLGRVGTKCCTLPEDQRLPCVEDYLSAILNRVCLLHEKTPVSEHVTKCCSGSLVERRPCFSALTVDETYVPKEFKAETFTFHSDICTLPEKEKQIKKQTALAELVKHKPKATAEQLKTVMDDFAQFLDTCCKAADKDTCFSTEGPNLVTRCKDALA

SEQ ID NO: 62 - protein, 1509 aa, Artificial Sequence
  ENPP5-ENPP3-Albumin
MTSKFLLVSFILAALSLSTTFSKQGSCRKKCFDASFRGLENCRCDVACKDRGDCCWDFEDTCVESTRIWMCNKFRCGERLEASLCSCSDDCLQRKDCCADYKSVCQGETSWLEENCDTAQQSQCPEGFDLPPVILFSMDGFRAEYLYTWDTLMPNINKLKTCGIHSKYMRAMYPTKTFPNHYTIVTGLYPESHGIIDNNMYDVNLNKNFSLSSKEQNNPAWWHGQPMWLTAMYQGLKAATYFWPGSEVAINGSFPSIYMPYNGSVPFEERISTLLKWLDLPKAERPRFYTMYFEEPDSSGHAGGPVSARVIKALQVVDHAFGMLMEGLKQRNLHNCVNIILLADHGMDQTYCNKMEYMTDYFPRINFFYMYEGPAPRIRAHNIPHDFFSFNSEEIVRNLSCRKPDQHFKPYLTPDLPKRLHYAKNVRIDKVHLFVDQQWLAVRSKSNTNCGGGNHGYNNEFRSMEAIFLAHGPSFKEKTEVEPFENIEVYNLMCDLLRIQPAPNNGTHGSLNHLLKVPFYEPSHAEEVSKFSVCGFANPLPTESLDCFCPHLQNSTQLEQVNQMLNLTQEEITATVKVNLPFGRPRVLQKNVDHCLLYHREYVSGFGKAMRMPMWSSYTVPQLGDTSPLPPTVPDCLRADVRVPPSESQKCSFYLADKNITHGFLYPPASNRTSDSQYDALITSNLVPMYEEFRKMWDYFHSVLLIKHATERNGVNVVSGPIFDYNYDGHFDAPDEITKHLANTDVPIPTHYFVVLTSCKNKSHTPENCPGWLDVLPFIIPHRPTNVESCPEGKPEALWVEERFTAHIARVRDVELLTGLDFYQDKVQPVSEILQLKTYLPTFETTIDKTHTCPPCPAPELLGGPSVFLFPPKPKDTLMISRTPEVTGGGSGGGGSGGGGSMKWVTFLLLLFVSGSAFSRGVFRREAHKSEIAHRYNDLGEQHFKGLVLIAFSQYLQKCSYDEHAKLVQEVTDFAKTCVADESAANCDKSLHTLFGDKLCAIPNLRENYGELADCCTKQEPERNECFLQHKDDNPSLPPFERPEAEAMCTSFKENPTTFMGHYLHEVARRHPYFYAPELLYYAEQYNEILTQCCAEADKESCLTPKLDGVKEKALVSSVRQRMKCSSMQKFGERAFKAWAVARLSQTFPNADFAEITKLATDLTKVNKECCHGDLLECADDRAELAKYMCENQATISSKLQTCCDKPLLKKAHCLSEVEHDTMPADLPAIAADFVEDQEVCKNYAEAKDVFLGTFLYEYSRRHPDYSVSLLLRLAKKYEATLEKCCAEANPPACYGTVLAEFQPLVEEPKNLVKTNCDLYEKLGEYGFQNAILVRYTQKAPQVSTPTLVEAARNLGRVGTKCCTLPEDQRLPCVEDYLSAILNRVCLLHEKTPVSEHVTKCCSGSLVERRPCFSALTVDETYVPKEFKAETFTFHSDICTLPEKEKQIKKQTALAELVKHKPKATAEQLKTVMDDFAQFLDTCCKAADKDTCFSTEGPNLVTRCKDALA

SEQ ID NO: 63 - DNA, 3447 bp, Artificial Sequence
  ENPP121-ENPP3-Fc nucleotide sequence
atggaaagggacggatgcgccggtggtggatctcgcggaggcgaaggtggaagggcccctagggaaggacctgccggaaacggaagggacaggggacgctctcacgccgctgaagctccaggcgaccctcaggccgctgcctctctgctggctcctatggacgtcggagaagaacccctggaaaaggccgccagggccaggactgccaaggaccccaacacctacaagatcatctccctcttcactttcgccgtcggagtcaacatctgcctgggattcaccgccgaaaagcaaggcagctgcaggaagaagtgctttgatgcatcatttagaggactggagaactgccggtgtgatgtggcatgtaaagaccgaggtgattgctgctgggattttgaagacacctgtgtggaatcaactcgaatatggatgtgcaataaatttcgttgtggagagaccagattagaggccagcctttgctcttgttcagatgactgtttgcagaggaaagattgctgtgctgactataagagtgtttgccaaggagaaacctcatggctggaagaaaactgtgacacagcccagcagtctcagtgcccagaagggtttgacctgccaccagttatcttgttttctatggatggatttagagctgaatatttatacacatgggatactttaatgccaaatatcaataaactgaaaacatgtggaattcattcaaaatacatgagagctatgtatcctaccaaaaccttcccaaatcattacaccattgtcacgggcttgtatccagagtcacatggcatcattgacaataatatgtatgatgtaaatctcaacaagaatttttcactttcttcaaaggaacaaaataatccagcctggtggcatgggcaaccaatgtggctgacagcaatgtatcaaggtttaaaagccgctacctacttttggcccggatcagaagtggctataaatggctcctttccttccatatacatgccttacaacggaagtgtcccatttgaagagaggatttctacactgttaaaatggctggacctgcccaaagctgaaagacccaggttttataccatgtattttgaagaacctgattcctctggacatgcaggtggaccagtcagtgccagagtaattaaagccttacaggtagtagatcatgcttttgggatgttgatggaaggcctgaagcagcggaatttgcacaactgtgtcaatatcatccttctggctgaccatggaatggaccagacttattgtaacaagatggaatacatgactgattattttcccagaataaacttcttctacatgtacgaagggcctgccccccgcatccgagctcataatatacctcatgacttttttagttttaattctgaggaaattgttagaaacctcagttgccgaaaacctgatcagcatttcaagccctatttgactcctgatttgccaaagcgactgcactatgccaagaacgtcagaatcgacaaagttcatctctttgtggatcaacagtggctggctgttaggagtaaatcaaatacaaattgtggaggaggcaaccatggttataacaatgagtttaggagcatggaggctatctttctggcacatggacccagttttaaagagaagactgaagttgaaccatttgaaaatattgaagtctataacctaatgtgtgatcttctacgcattcaaccagcaccaaacaatggaacccatggtagtttaaaccatcttctgaaggtgcctttttatgagccatcccatgcagaggaggtgtcaaagttttctgtttgtggctttgctaatccattgcccacagagtctcttgactgtttctgccctcacctacaaaatagtactcagctggaacaagtgaatcagatgctaaatctcacccaagaagaaataacagcaacagtgaaagtaaatttgccatttgggaggcctagggtactgcagaagaacgtggaccactgtctcctttaccacagggaatatgtcagtggatttggaaaagctatgaggatgcccatgtggagttcatacacagtcccccagttgggagacacatcgcctctgcctcccactgtcccagactgtctgcgggctgatgtcagggttcctccttctgagagccaaaaatgttccttctatttagcagacaagaatatcacccacggcttcctctatcctcctgccagcaatagaacatcagatagccaatatgatgctttaattactagcaatttggtacctatgtatgaagaattcagaaaaatgtgggactacttccacagtgttcttcttataaaacatgccacagaaagaaatggagtaaatgtggttagtggaccaatatttgattataattatgatggccattttgatgctccagatgaaattaccaaacatttagccaacactgatgttcccatcccaacacactactttgtggtgctgaccagttgtaaaaacaagagccacacaccggaaaactgccctgggtggctggatgtcctaccctttatcatccctcaccgacctaccaacgtggagagctgtcctgaaggtaaaccagaagctctttgggttgaagaaagatttacagctcacattgcccgggtccgtgatgtagaacttctcactgggcttgacttctatcaggataaagtgcagcctgtctctgaaattttgcaactaaagacatatttaccaacatttgaaaccactattgacaaaactcacacatgcccaccgtgcccagcacctgaactcctggggggaccgtcagtcttcctcttccccccaaaacccaaggacaccctcatgatctcccggacccctgaggtcacatgcgtggtggtggacgtgagccacgaagaccctgaggtcaagttcaactggtacgtggacggcgtggaggtgcataatgccaagacaaagccgcgggaggagcagtacaacagcacgtaccgtgtggtcagcgtcctcaccgtcctgcaccaggactggctgaatggcaaggagtacaagtgcaaggtctccaacaaagccctcccagcccccatcgagaaaaccatctccaaagccaaagggcagccccgagaaccacaggtgtacaccctgcccccatcccgggaggagatgaccaagaaccaggtcagcctgacctgcctggtcaaaggcttctatcccagcgacatcgccgtggagtgggagagcaatgggcagccggagaacaactacaagaccacgcctcccgtgctggactccgacggctccttcttcctctatagcaagctcaccgtggacaagagcaggtggcagcaggggaacgtcttctcatgctccgtgatgcatgaggctctgcacaaccactacacgcagaagagcctctccctgtccccgggtaaa

SEQ ID NO: 64 - DNA, 4638 bp, Artificial Sequence
  ENPP121-ENPP3-Albumin nucleotide sequence
atggaaagggacggatgcgccggtggtggatctcgcggaggcgaaggtggaagggcccctagggaaggacctgccggaaacggaagggacaggggacgctctcacgccgctgaagctccaggcgaccctcaggccgctgcctctctgctggctcctatggacgtcggagaagaacccctggaaaaggccgccagggccaggactgccaaggaccccaacacctacaagatcatctccctcttcactttcgccgtcggagtcaacatctgcctgggattcaccgccgaaaagcaaggcagctgcaggaagaagtgctttgatgcatcatttagaggactggagaactgccggtgtgatgtggcatgtaaagaccgaggtgattgctgctgggattttgaagacacctgtgtggaatcaactcgaatatggatgtgcaataaatttcgttgtggagagaccagattagaggccagcctttgctcttgttcagatgactgtttgcagaggaaagattgctgtgctgactataagagtgtttgccaaggagaaacctcatggctggaagaaaactgtgacacagcccagcagtctcagtgcccagaagggtttgacctgccaccagttatcttgttttctatggatggatttagagctgaatatttatacacatgggatactttaatgccaaatatcaataaactgaaaacatgtggaattcattcaaaatacatgagagctatgtatcctaccaaaaccttcccaaatcattacaccattgtcacgggcttgtatccagagtcacatggcatcattgacaataatatgtatgatgtaaatctcaacaagaatttttcactttcttcaaaggaacaaaataatccagcctggtggcatgggcaaccaatgtggctgacagcaatgtatcaaggtttaaaagccgctacctacttttggcccggatcagaagtggctataaatggctcctttccttccatatacatgccttacaacggaagtgtcccatttgaagagaggatttctacactgttaaaatggctggacctgcccaaagctgaaagacccaggttttataccatgtattttgaagaacctgattcctctggacatgcaggtggaccagtcagtgccagagtaattaaagccttacaggtagtagatcatgcttttgggatgttgatggaaggcctgaagcagcggaatttgcacaactgtgtcaatatcatccttctggctgaccatggaatggaccagacttattgtaacaagatggaatacatgactgattattttcccagaataaacttcttctacatgtacgaagggcctgccccccgcatccgagctcataatatacctcatgacttttttagttttaattctgaggaaattgttagaaacctcagttgccgaaaacctgatcagcatttcaagccctatttgactcctgatttgccaaagcgactgcactatgccaagaacgtcagaatcgacaaagttcatctctttgtggatcaacagtggctggctgttaggagtaaatcaaatacaaattgtggaggaggcaaccatggttataacaatgagtttaggagcatggaggctatctttctggcacatggacccagttttaaagagaagactgaagttgaaccatttgaaaatattgaagtctataacctaatgtgtgatcttctacgcattcaaccagcaccaaacaatggaacccatggtagtttaaaccatcttctgaaggtgcctttttatgagccatcccatgcagaggaggtgtcaaagttttctgtttgtggctttgctaatccattgcccacagagtctcttgactgtttctgccctcacctacaaaatagtactcagctggaacaagtgaatcagatgctaaatctcacccaagaagaaataacagcaacagtgaaagtaaatttgccatttgggaggcctagggtactgcagaagaacgtggaccactgtctcctttaccacagggaatatgtcagtggatttggaaaagctatgaggatgcccatgtggagttcatacacagtcccccagttgggagacacatcgcctctgcctcccactgtcccagactgtctgcgggctgatgtcagggttcctccttctgagagccaaaaatgttccttctatttagcagacaagaatatcacccacggcttcctctatcctcctgccagcaatagaacatcagatagccaatatgatgctttaattactagcaatttggtacctatgtatgaagaattcagaaaaatgtgggactacttccacagtgttcttcttataaaacatgccacagaaagaaatggagtaaatgtggttagtggaccaatatttgattataattatgatggccattttgatgctccagatgaaattaccaaacatttagccaacactgatgttcccatcccaacacactactttgtggtgctgaccagttgtaaaaacaagagccacacaccggaaaactgccctgggtggctggatgtcctaccctttatcatccctcaccgacctaccaacgtggagagctgtcctgaaggtaaaccagaagctctttgggttgaagaaagatttacagctcacattgcccgggtccgtgatgtagaacttctcactgggcttgacttctatcaggataaagtgcagcctgtctctgaaattttgcaactaaagacatatttaccaacatttgaaaccactattggtggaggaggctctggtggaggcggtagcggaggcggagggtcgatgaagtgggtaacctttatttcccttctttttctctttagctcggcttattccaggggtgtgtttcgtcgagatgcacacaagagtgaggttgctcatcggtttaaagatttgggagaagaaaatttcaaagccttggtgttgattgcctttgctcagtatcttcagcagtgtccatttgaagatcatgtaaaattagtgaatgaagtaactgaatttgcaaaaacatgtgttgctgatgagtcagctgaaaattgtgacaaatcacttcataccctttttggagacaaattatgcacagttgcaactcttcgtgaaacctatggtgaaatggctgactgctgtgcaaaacaagaacctgagagaaatgaatgcttcttgcaacacaaagatgacaacccaaacctcccccgattggtgagaccagaggttgatgtgatgtgcactgcttttcatgacaatgaagagacatttttgaaaaaatacttatatgaaattgccagaagacatccttacttttatgccccggaactccttttctttgctaaaaggtataaagctgcttttacagaatgttgccaagctgctgataaagctgcctgcctgttgccaaagctcgatgaacttcgggatgaagggaaggcttcgtctgccaaacagagactcaagtgtgccagtctccaaaaatttggagaaagagctttcaaagcatgggcagtagctcgcctgagccagagatttcccaaagctgagtttgcagaagtttccaagttagtgacagatcttaccaaagtccacacggaatgctgccatggagatctgcttgaatgtgctgatgacagggcggaccttgccaagtatatctgtgaaaatcaagattcgatctccagtaaactgaaggaatgctgtgaaaaacctctgttggaaaaatcccactgcattgccgaagtggaaaatgatgagatgcctgctgacttgccttcattagctgctgattttgttgaaagtaaggatgtttgcaaaaactatgctgaggcaaaggatgtcttcctgggcatgtttttgtatgaatatgcaagaaggcatcctgattactctgtcgtgctgctgctgagacttgccaagacatatgaaaccactctagagaagtgctgtgccgctgcagatcctcatgaatgctatgccaaagtgttcgatgaatttaaacctcttgtggaagagcctcagaatttaatcaaacaaaattgtgagctttttgagcagcttggagagtacaaattccagaatgcgctattagttcgttacaccaagaaagtaccccaagtgtcaactccaactcttgtagaggtctcaagaaacctaggaaaagtgggcagcaaatgttgtaaacatcctgaagcaaaaagaatgccctgtgcagaagactatctatccgtggtcctgaaccagttatgtgtgttgcatgagaaaacgccagtaagtgacagagtcaccaaatgctgcacagaatccttggtgaacaggcgaccatgcttttcagctctggaagtcgatgaaacatacgttcccaaagagtttaatgctgaaacattcaccttccatgcagatatatgcacactttctgagaaggagagacaaatcaagaaacaaactgcacttgttgagctcgtgaaacacaagcccaaggcaacaaaagagcaactgaaagctgttatggatgatttcgcagcttttgtagagaagtgctgcaaggctgacgataaggagacctgctttgccgaggagggtaaaaaacttgttgctgcaagtcaagctgccttaggctta

SEQ ID NO: 65 - DNA, 8852 bp, Artificial Sequence
  hNPP3-hFc-pcDNA3 nucleotide sequence
gacggatcgggagatctcccgatcccctatggtcgactctcagtacaatctgctctgatgccgcatagttaagccagtatctgctccctgcttgtgtgttggaggtcgctgagtagtgcgcgagcaaaatttaagctacaacaaggcaaggcttgaccgacaattgcatgaagaatctgcttagggttaggcgttttgcgctgcttcgcgatgtacgggccagatatacgcgttgacattgattattgactagttattaatagtaatcaattacggggtcattagttcatagcccatatatggagttccgcgttacataacttacggtaaatggcccgcctggctgaccgcccaacgacccccgcccattgacgtcaataatgacgtatgttcccatagtaacgccaatagggactttccattgacgtcaatgggtggactatttacggtaaactgcccacttggcagtacatcaagtgtatcatatgccaagtacgccccctattgacgtcaatgacggtaaatggcccgcctggcattatgcccagtacatgaccttatgggactttcctacttggcagtacatctacgtattagtcatcgctattaccatggtgatgcggttttggcagtacatcaatgggcgtggatagcggtttgactcacggggatttccaagtctccaccccattgacgtcaatgggagtttgttttggcaccaaaatcaacgggactttccaaaatgtcgtaacaactccgccccattgacgcaaatgggcggtaggcgtgtacggtgggaggtctatataagcagagctctctggctaactagagaacccactgcttactggcttatcgaaattaatacgactcactatagggagacccaagcttatggaaagggacggatgcgccggtggtggatctcgcggaggcgaaggtggaagggcccctagggaaggacctgccggaaacggaagggacaggggacgctctcacgccgctgaagctccaggcgaccctcaggccgctgcctctctgctggctcctatggacgtcggagaagaacccctggaaaaggccgccagggccaggactgccaaggaccccaacacctacaagatcatctccctcttcactttcgccgtcggagtcaacatctgcctgggattcaccgccgaaaagcaaggcagctgcaggaagaagtgctttgatgcatcatttagaggactggagaactgccggtgtgatgtggcatgtaaagaccgaggtgattgctgctgggattttgaagacacctgtgtggaatcaactcgaatatggatgtgcaataaatttcgttgtggagagaccagattagaggccagcctttgctcttgttcagatgactgtttgcagaggaaagattgctgtgctgactataagagtgtttgccaaggagaaacctcatggctggaagaaaactgtgacacagcccagcagtctcagtgcccagaagggtttgacctgccaccagttatcttgttttctatggatggatttagagctgaatatttatacacatgggatactttaatgccaaatatcaataaactgaaaacatgtggaattcattcaaaatacatgagagctatgtatcctaccaaaaccttcccaaatcattacaccattgtcacgggcttgtatccagagtcacatggcatcattgacaataatatgtatgatgtaaatctcaacaagaatttttcactttcttcaaaggaacaaaataatccagcctggtggcatgggcaaccaatgtggctgacagcaatgtatcaaggtttaaaagccgctacctacttttggcccggatcagaagtggctataaatggctcctttccttccatatacatgccttacaacggaagtgtcccatttgaagagaggatttctacactgttaaaatggctggacctgcccaaagctgaaagacccaggttttataccatgtattttgaagaacctgattcctctggacatgcaggtggaccagtcagtgccagagtaattaaagccttacaggtagtagatcatgcttttgggatgttgatggaaggcctgaagcagcggaatttgcacaactgtgtcaatatcatccttctggctgaccatggaatggaccagacttattgtaacaagatggaatacatgactgattattttcccagaataaacttcttctacatgtacgaagggcctgccccccgcatccgagctcataatatacctcatgacttttttagttttaattctgaggaaattgttagaaacctcagttgccgaaaacctgatcagcatttcaagccctatttgactcctgatttgccaaagcgactgcactatgccaagaacgtcagaatcgacaaagttcatctctttgtggatcaacagtggctggctgttaggagtaaatcaaatacaaattgtggaggaggcaaccatggttataacaatgagtttaggagcatggaggctatctttctggcacatggacccagttttaaagagaagactgaagttgaaccatttgaaaatattgaagtctataacctaatgtgtgatcttctacgcattcaaccagcaccaaacaatggaacccatggtagtttaaaccatcttctgaaggtgcctttttatgagccatcccatgcagaggaggtgtcaaagttttctgtttgtggctttgctaatccattgcccacagagtctcttgactgtttctgccctcacctacaaaatagtactcagctggaacaagtgaatcagatgctaaatctcacccaagaagaaataacagcaacagtgaaagtaaatttgccatttgggaggcctagggtactgcagaagaacgtggaccactgtctcctttaccacagggaatatgtcagtggatttggaaaagctatgaggatgcccatgtggagttcatacacagtcccccagttgggagacacatcgcctctgcctcccactgtcccagactgtctgcgggctgatgtcagggttcctccttctgagagccaaaaatgttccttctatttagcagacaagaatatcacccacggcttcctctatcctcctgccagcaatagaacatcagatagccaatatgatgctttaattactagcaatttggtacctatgtatgaagaattcagaaaaatgtgggactacttccacagtgttcttcttataaaacatgccacagaaagaaatggagtaaatgtggttagtggaccaatatttgattataattatgatggccattttgatgctccagatgaaattaccaaacatttagccaacactgatgttcccatcccaacacactactttgtggtgctgaccagttgtaaaaacaagagccacacaccggaaaactgccctgggtggctggatgtcctaccctttatcatccctcaccgacctaccaacgtggagagctgtcctgaaggtaaaccagaagctctttgggttgaagaaagatttacagctcacattgcccgggtccgtgatgtagaacttctcactgggcttgacttctatcaggataaagtgcagcctgtctctgaaattttgcaactaaagacatatttaccaacatttgaaaccactattgacaaaactcacacatgcccaccgtgcccagcacctgaactcctggggggaccgtcagtcttcctcttccccccaaaacccaaggacaccctcatgatctcccggacccctgaggtcacatgcgtggtggtggacgtgagccacgaagaccctgaggtcaagttcaactggtacgtggacggcgtggaggtgcataatgccaagacaaagccgcgggaggagcagtacaacagcacgtaccgtgtggtcagcgtcctcaccgtcctgcaccaggactggctgaatggcaaggagtacaagtgcaaggtctccaacaaagccctcccagcccccatcgagaaaaccatctccaaagccaaagggcagccccgagaaccacaggtgtacaccctgcccccatcccgggaggagatgaccaagaaccaggtcagcctgacctgcctggtcaaaggcttctatcccagcgacatcgccgtggagtgggagagcaatgggcagccggagaacaactacaagaccacgcctcccgtgctggactccgacggctccttcttcctctatagcaagctcaccgtggacaagagcaggtggcagcaggggaacgtcttctcatgctccgtgatgcatgaggctctgcacaaccactacacgcagaagagcctctccctgtccccgggtaaatgaaattctgcagatatccatcacactggcggccgctcgagcatgcatctagagggccctattctatagtgtcacctaaatgctagagctcgctgatcagcctcgactgtgccttctagttgccagccatctgttgtttgcccctcccccgtgccttccttgaccctggaaggtgccactcccactgtcctttcctaataaaatgaggaaattgcatcgcattgtctgagtaggtgtcattctattctggggggtggggtggggcaggacagcaagggggaggattgggaagacaatagcaggcatgctggggatgcggtgggctctatggcttctgaggcggaaagaaccagctggggctctagggggtatccccacgcgccctgtagcggcgcattaagcgcggcgggtgtggtggttacgcgcagcgtgaccgctacacttgccagcgccctagcgcccgctcctttcgctttcttcccttcctttctcgccacgttcgccggctttccccgtcaagctctaaatcggggcatccctttagggttccgatttagtgctttacggcacctcgaccccaaaaaacttgattagggtgatggttcacgtagtgggccatcgccctgatagacggtttttcgccctttgacgttggagtccacgttctttaatagtggactcttgttccaaactggaacaacactcaaccctatctcggtctattcttttgatttataagggattttggggatttcggcctattggttaaaaaatgagctgatttaacaaaaatttaacgcgaattaattctgtggaatgtgtgtcagttagggtgtggaaagtccccaggctccccaggcaggcagaagtatgcaaagcatgcatctcaattagtcagcaaccaggtgtggaaagtccccaggctccccagcaggcagaagtatgcaaagcatgcatctcaattagtcagcaaccatagtcccgcccctaactccgcccatcccgcccctaactccgcccagttccgcccattctccgccccatggctgactaattttttttatttatgcagaggccgaggccgcctctgcctctgagctattccagaagtagtgaggaggcttttttggaggcctaggcttttgcaaaaagctcccgggagcttgtatatccattttcggatctgatcaagagacaggatgaggatcgtttcgcatgattgaacaagatggattgcacgcaggttctccggccgcttgggtggagaggctattcggctatgactgggcacaacagacaatcggctgctctgatgccgccgtgttccggctgtcagcgcaggggcgcccggttctttttgtcaagaccgacctgtccggtgccctgaatgaactgcaggacgaggcagcgcggctatcgtggctggccacgacgggcgttccttgcgcagctgtgctcgacgttgtcactgaagcgggaagggactggctgctattgggcgaagtgccggggcaggatctcctgtcatctcaccttgctcctgccgagaaagtatccatcatggctgatgcaatgcggcggctgcatacgcttgatccggctacctgcccattcgaccaccaagcgaaacatcgcatcgagcgagcacgtactcggatggaagccggtcttgtcgatcaggatgatctggacgaagagcatcaggggctcgcgccagccgaactgttcgccaggctcaaggcgcgcatgcccgacggcgaggatctcgtcgtgacccatggcgatgcctgcttgccgaatatcatggtggaaaatggccgcttttctggattcatcgactgtggccggctgggtgtggcggaccgctatcaggacatagcgttggctacccgtgatattgctgaagagcttggcggcgaatgggctgaccgcttcctcgtgctttacggtatcgccgctcccgattcgcagcgcatcgccttctatcgccttcttgacgagttcttctgagcgggactctggggttcgaaatgaccgaccaagcgacgcccaacctgccatcacgagatttcgattccaccgccgccttctatgaaaggttgggcttcggaatcgttttccgggacgccggctggatgatcctccagcgcggggatctcatgctggagttcttcgcccaccccaacttgtttattgcagcttataatggttacaaataaagcaatagcatcacaaatttcacaaataaagcatttttttcactgcattctagttgtggtttgtccaaactcatcaatgtatcttatcatgtctgtataccgtcgacctctagctagagcttggcgtaatcatggtcatagctgtttcctgtgtgaaattgttatccgctcacaattccacacaacatacgagccggaagcataaagtgtaaagcctggggtgcctaatgagtgagctaactcacattaattgcgttgcgctcactgcccgctttccagtcgggaaacctgtcgtgccagctgcattaatgaatcggccaacgcgcggggagaggcggtttgcgtattgggcgctcttccgcttcctcgctcactgactcgctgcgctcggtcgttcggctgcggcgagcggtatcagctcactcaaaggcggtaatacggttatccacagaatcaggggataacgcaggaaagaacatgtgagcaaaaggccagcaaaaggccaggaaccgtaaaaaggccgcgttgctggcgtttttccataggctccgcccccctgacgagcatcacaaaaatcgacgctcaagtcagaggtggcgaaacccgacaggactataaagataccaggcgtttccccctggaagctccctcgtgcgctctcctgttccgaccctgccgcttaccggatacctgtccgcctttctcccttcgggaagcgtggcgctttctcaatgctcacgctgtaggtatctcagttcggtgtaggtcgttcgctccaagctgggctgtgtgcacgaaccccccgttcagcccgaccgctgcgccttatccggtaactatcgtcttgagtccaacccggtaagacacgacttatcgccactggcagcagccactggtaacaggattagcagagcgaggtatgtaggcggtgctacagagttcttgaagtggtggcctaactacggctacactagaaggacagtatttggtatctgcgctctgctgaagccagttaccttcggaaaaagagttggtagctcttgatccggcaaacaaaccaccgctggtagcggtggtttttttgtttgcaagcagcagattacgcgcagaaaaaaaggatctcaagaagatcctttgatcttttctacggggtctgacgctcagtggaacgaaaactcacgttaagggattttggtcatgagattatcaaaaaggatcttcacctagatccttttaaattaaaaatgaagttttaaatcaatctaaagtatatatgagtaaacttggtctgacagttaccaatgcttaatcagtgaggcacctatctcagcgatctgtctatttcgttcatccatagttgcctgactccccgtcgtgtagataactacgatacgggagggcttaccatctggccccagtgctgcaatgataccgcgagacccacgctcaccggctccagatttatcagcaataaaccagccagccggaagggccgagcgcagaagtggtcctgcaactttatccgcctccatccagtctattaattgttgccgggaagctagagtaagtagttcgccagttaatagtttgcgcaacgttgttgccattgctacaggcatcgtggtgtcacgctcgtcgtttggtatggcttcattcagctccggttcccaacgatcaaggcgagttacatgatcccccatgttgtgcaaaaaagcggttagctccttcggtcctccgatcgttgtcagaagtaagttggccgcagtgttatcactcatggttatggcagcactgcataattctcttactgtcatgccatccgtaagatgcttttctgtgactggtgagtactcaaccaagtcattctgagaatagtgtatgcggcgaccgagttgctcttgcccggcgtcaatacgggataataccgcgccacatagcagaactttaaaagtgctcatcattggaaaacgttcttcggggcgaaaactctcaaggatcttaccgctgttgagatccagttcgatgtaacccactcgtgcacccaactgatcttcagcatcttttactttcaccagcgtttctgggtgagcaaaaacaggaaggcaaaatgccgcaaaaaagggaataagggcgacacggaaatgttgaatactcatactcttcctttttcaatattattgaagcatttatcagggttattgtctcatgagcggatacatatttgaatgtatttagaaaaataaacaaataggggttccgcgcacatttccccgaaaagtgccacctgacgtc

SEQ ID NO: 66 - protein, 1152 aa, Artificial Sequence
  ENPP121-Fc
MERDGCAGGGSRGGEGGRAPREGPAGNGRDRGRSHAAEAPGDPQAAASLLAPMDVGEEPLEKAARARTAKDPNTYKIISLFTFAVGVNICLGFTAGLKPSCAKEVKSCKGRCFERTFGNCRCDAACVELGNCCLDYQETCIEPEHIWTCNKFRCGEKRLTRSLCACSDDCKDKGDCCINYSSVCQGEKSWVEEPCESINEPQCPAGFETPPTLLFSLDGFRAEYLHTWGGLLPVISKLKKCGTYTKNMRPVYPTKTFPNHYSIVTGLYPESHGIIDNKMYDPKMNASFSLKSKEKFNPEWYKGEPIWVTAKYQGLKSGTFFWPGSDVEINGIFPDIYKMYNGSVPFEERILAVLQWLQLPKDERPHFYTLYLEEPDSSGHSYGPVSSEVIKALQRVDGMVGMLMDGLKELNLHRCLNLILISDHGMEQGSCKKYIYLNKYLGDVKNIKVIYGPAARLRPSDVPDKYYSFNYEGIARNLSCREPNQHFKPYLKHFLPKRLHFAKSDRIEPLTFYLDPQWQLALNPSERKYCGSGFHGSDNVFSNMQALFVGYGPGFKHGIEADTFENIEVYNLMCDLLNLTPAPNNGTHGSLNHLLKNPVYTPKHPKEVHPLVQCPFTRNPRDNLGCSCNPSILPIEDFQTQFNLTVAEEKIIKHETLPYGRPRVLQKENTICLLSQHQFMSGYSQDILMPLWTSYTVDRNDSFSTEDFSNCLYQDFRIPLSPVHKCSFYKNNTKVSYGFLSPPQLNKNSSGIYSEALLTTNIVPMYQSFQVIWRYFHDTLLRKYAEERNGVNVVSGPVFDFDYDGRCDSLENLRQKRRVIRNQEILIPTHFFIVLTSCKDTSQTPLHCENLDTLAFILPHRTDNSESCVHGKHDSSWVEELLMLHRARITDVEHITGLSFYQQRKEPVSDILKLKTHLPTFSQEDDKTHTCPPCPAPELLGGPSVFLFPPKPKDTLMISRTPEVTCVVVDVSHEDPEVKFNWYVDGVEVHNAKTKPREEQYNSTYRVVSVLTVLHQDWLNGKEYKCKVSNKALPAPIEKTISKAKGQPREPQVYTLPPSREEMTKNQVSLTCLVKGFYPSDIAVEWESNGQPENNYKTTPPVLDSDGSFFLYSKLTVDKSRWQQGNVFSCSVMHEALHNHYTQKSLSLSPGK

SEQ ID NO: 67 - protein, 1077 aa, Artificial Sequence
  ENPP71-Fc
MRGPAVLLTVALATLLAPGAGLKPSCAKEVKSCKGRCFERTFGNCRCDAACVELGNCCLDYQETCIEPEHIWTCNKFRCGEKRLTRSLCACSDDCKDKGDCCINYSSVCQGEKSWVEEPCESINEPQCPAGFETPPTLLFSLDGFRAEYLHTWGGLLPVISKLKKCGTYTKNMRPVYPTKTFPNHYSIVTGLYPESHGIIDNKMYDPKMNASFSLKSKEKFNPEWYKGEPIWVTAKYQGLKSGTFFWPGSDVEINGIFPDIYKMYNGSVPFEERILAVLQWLQLPKDERPHFYTLYLEEPDSSGHSYGPVSSEVIKALQRVDGMVGMLMDGLKELNLHRCLNLILISDHGMEQGSCKKYIYLNKYLGDVKNIKVIYGPAARLRPSDVPDKYYSFNYEGIARNLSCREPNQHFKPYLKHFLPKRLHFAKSDRIEPLTFYLDPQWQLALNPSERKYCGSGFHGSDNVFSNMQALFVGYGPGFKHGIEADTFENIEVYNLMCDLLNLTPAPNNGTHGSLNHLLKNPVYTPKHPKEVHPLVQCPFTRNPRDNLGCSCNPSILPIEDFQTQFNLTVAEEKIIKHETLPYGRPRVLQKENTICLLSQHQFMSGYSQDILMPLWTSYTVDRNDSFSTEDFSNCLYQDFRIPLSPVHKCSFYKNNTKVSYGFLSPPQLNKNSSGIYSEALLTTNIVPMYQSFQVIWRYFHDTLLRKYAEERNGVNVVSGPVFDFDYDGRCDSLENLRQKRRVIRNQEILIPTHFFIVLTSCKDTSQTPLHCENLDTLAFILPHRTDNSESCVHGKHDSSWVEELLMLHRARITDVEHITGLSFYQQRKEPVSDILKLKTHLPTFSQEDDKTHTCPPCPAPELLGGPSVFLFPPKPKDTLMISRTPEVTCVVVDVSHEDPEVKFNWYVDGVEVHNAKTKPREEQYNSTYRVVSVLTVLHQDWLNGKEYKCKVSNKALPAPIEKTISKAKGQPREPQVYTLPPSREEMTKNQVSLTCLVKGFYPSDIAVEWESNGQPENNYKTTPPVLDSDGSFFLYSKLTVDKSRWQQGNVFSCSVMHEALHNHYTQKSLSLSPGK

SEQ ID NO: 68 - protein, 1079 aa, Artificial Sequence
  ENPP51-Fc
MTSKFLLVSFILAALSLSTTFSGLKPSCAKEVKSCKGRCFERTFGNCRCDAACVELGNCCLDYQETCIEPEHIWTCNKFRCGEKRLTRSLCACSDDCKDKGDCCINYSSVCQGEKSWVEEPCESINEPQCPAGFETPPTLLFSLDGFRAEYLHTWGGLLPVISKLKKCGTYTKNMRPVYPTKTFPNHYSIVTGLYPESHGIIDNKMYDPKMNASFSLKSKEKFNPEWYKGEPIWVTAKYQGLKSGTFFWPGSDVEINGIFPDIYKMYNGSVPFEERILAVLQWLQLPKDERPHFYTLYLEEPDSSGHSYGPVSSEVIKALQRVDGMVGMLMDGLKELNLHRCLNLILISDHGMEQGSCKKYIYLNKYLGDVKNIKVIYGPAARLRPSDVPDKYYSFNYEGIARNLSCREPNQHFKPYLKHFLPKRLHFAKSDRIEPLTFYLDPQWQLALNPSERKYCGSGFHGSDNVFSNMQALFVGYGPGFKHGIEADTFENIEVYNLMCDLLNLTPAPNNGTHGSLNHLLKNPVYTPKHPKEVHPLVQCPFTRNPRDNLGCSCNPSILPIEDFQTQFNLTVAEEKIIKHETLPYGRPRVLQKENTICLLSQHQFMSGYSQDILMPLWTSYTVDRNDSFSTEDFSNCLYQDFRIPLSPVHKCSFYKNNTKVSYGFLSPPQLNKNSSGIYSEALLTTNIVPMYQSFQVIWRYFHDTLLRKYAEERNGVNVVSGPVFDFDYDGRCDSLENLRQKRRVIRNQEILIPTHFFIVLTSCKDTSQTPLHCENLDTLAFILPHRTDNSESCVHGKHDSSWVEELLMLHRARITDVEHITGLSFYQQRKEPVSDILKLKTHLPTFSQEDDKTHTCPPCPAPELLGGPSVFLFPPKPKDTLMISRTPEVTCVVVDVSHEDPEVKFNWYVDGVEVHNAKTKPREEQYNSTYRVVSVLTVLHQDWLNGKEYKCKVSNKALPAPIEKTISKAKGQPREPQVYTLPPSREEMTKNQVSLTCLVKGFYPSDIAVEWESNGQPENNYKTTPPVLDSDGSFFLYSKLTVDKSRWQQGNVFSCSVMHEALHNHYTQKSLSLSPGK

SEQ ID NO: 69 - protein, 1472 aa, Artificial Sequence
  ENPP121-ALB
MERDGCAGGGSRGGEGGRAPREGPAGNGRDRGRSHAAEAPGDPQAAASLLAPMDVGEEPLEKAARARTAKDPNTYKIISLFTFAVGVNICLGFTAGLKPSCAKEVKSCKGRCFERTFGNCRCDAACVELGNCCLDYQETCIEPEHIWTCNKFRCGEKRLTRSLCACSDDCKDKGDCCINYSSVCQGEKSWVEEPCESINEPQCPAGFETPPTLLFSLDGFRAEYLHTWGGLLPVISKLKKCGTYTKNMRPVYPTKTFPNHYSIVTGLYPESHGIIDNKMYDPKMNASFSLKSKEKFNPEWYKGEPIWVTAKYQGLKSGTFFWPGSDVEINGIFPDIYKMYNGSVPFEERILAVLQWLQLPKDERPHFYTLYLEEPDSSGHSYGPVSSEVIKALQRVDGMVGMLMDGLKELNLHRCLNLILISDHGMEQGSCKKYIYLNKYLGDVKNIKVIYGPAARLRPSDVPDKYYSFNYEGIARNLSCREPNQHFKPYLKHFLPKRLHFAKSDRIEPLTFYLDPQWQLALNPSERKYCGSGFHGSDNVFSNMQALFVGYGPGFKHGIEADTFENIEVYNLMCDLLNLTPAPNNGTHGSLNHLLKNPVYTPKHPKEVHPLVQCPFTRNPRDNLGCSCNPSILPIEDFQTQFNLTVAEEKIIKHETLPYGRPRVLQKENTICLLSQHQFMSGYSQDILMPLWTSYTVDRNDSFSTEDFSNCLYQDFRIPLSPVHKCSFYKNNTKVSYGFLSPPQLNKNSSGIYSEALLTTNIVPMYQSFQVIWRYFHDTLLRKYAEERNGVNVVSGPVFDFDYDGRCDSLENLRQKRRVIRNQEILIPTHFFIVLTSCKDTSQTPLHCENLDTLAFILPHRTDNSESCVHGKHDSSWVEELLMLHRARITDVEHITGLSFYQQRKEPVSDILKLKTHLPTFSQEDRSGSGGSMKWVTFLLLLFVSGSAFSRGVFRREAHKSEIAHRYNDLGEQHFKGLVLIAFSQYLQKCSYDEHAKLVQEVTDFAKTCVADESAANCDKSLHTLFGDKLCAIPNLRENYGELADCCTKQEPERNECFLQHKDDNPSLPPFERPEAEAMCTSFKENPTTFMGHYLHEVARRHPYFYAPELLYYAEQYNEILTQCCAEADKESCLTPKLDGVKEKALVSSVRQRMKCSSMQKFGERAFKAWAVARLSQTFPNADFAEITKLATDLTKVNKECCHGDLLECADDRAELAKYMCENQATISSKLQTCCDKPLLKKAHCLSEVEHDTMPADLPAIAADFVEDQEVCKNYAEAKDVFLGTFLYEYSRRHPDYSVSLLLRLAKKYEATLEKCCAEANPPACYGTVLAEFQPLVEEPKNLVKTNCDLYEKLGEYGFQNAILVRYTQKAPQVSTPTLVEAARNLGRVGTKCCTLPEDQRLPCVEDYLSAILNRVCLLHEKTPVSEHVTKCCSGSLVERRPCFSALTVDETYVPKEFKAETFTFHSDICTL

SEQ ID NO: 70 - protein, 1396 aa, Artificial Sequence
  NPP71-ALB
MRGPAVLLTVALATLLAPGAGLKPSCAKEVKSCKGRCFERTFGNCRCDAACVELGNCCLDYQETCIEPEHIWTCNKFRCGEKRLTRSLCACSDDCKDKGDCCINYSSVCQGEKSWVEEPCESINEPQCPAGFETPPTLLFSLDGFRAEYLHTWGGLLPVISKLKKCGTYTKNMRPVYPTKTFPNHYSIVTGLYPESHGIIDNKMYDPKMNASFSLKSKEKFNPEWYKGEPIWVTAKYQGLKSGTFFWPGSDVEINGIFPDIYKMYNGSVPFEERILAVLQWLQLPKDERPHFYTLYLEEPDSSGHSYGPVSSEVIKALQRVDGMVGMLMDGLKELNLHRCLNLILISDHGMEQGSCKKYIYLNKYLGDVKNIKVIYGPAARLRPSDVPDKYYSFNYEGIARNLSCREPNQHFKPYLKHFLPKRLHFAKSDRIEPLTFYLDPQWQLALNPSERKYCGSGFHGSDNVFSNMQALFVGYGPGFKHGIEADTFENIEVYNLMCDLLNLTPAPNNGTHGSLNHLLKNPVYTPKHPKEVHPLVQCPFTRNPRDNLGCSCNPSILPIEDFQTQFNLTVAEEKIIKHETLPYGRPRVLQKENTICLLSQHQFMSGYSQDILMPLWTSYTVDRNDSFSTEDFSNCLYQDFRIPLSPVHKCSFYKNNTKVSYGFLSPPQLNKNSSGIYSEALLTTNIVPMYQSFQVIWRYFHDTLLRKYAEERNGVNVVSGPVFDFDYDGRCDSLENLRQKRRVIRNQEILIPTHFFIVLTSCKDTSQTPLHCENLDTLAFILPHRTDNSESCVHGKHDSSWVEELLMLHRARITDVEHITGLSFYQQRKEPVSDILKLKTHLPTFSQEDGGSGGSMKWVTFLLLLFVSGSAFSRGVFRREAHKSEIAHRYNDLGEQHFKGLVLIAFSQYLQKCSYDEHAKLVQEVTDFAKTCVADESAANCDKSLHTLFGDKLCAIPNLRENYGELADCCTKQEPERNECFLQHKDDNPSLPPFERPEAEAMCTSFKENPTTFMGHYLHEVARRHPYFYAPELLYYAEQYNEILTQCCAEADKESCLTPKLDGVKEKALVSSVRQRMKCSSMQKFGERAFKAWAVARLSQTFPNADFAEITKLATDLTKVNKECCHGDLLECADDRAELAKYMCENQATISSKLQTCCDKPLLKKAHCLSEVEHDTMPADLPAIAADFVEDQEVCKNYAEAKDVFLGTFLYEYSRRHPDYSVSLLLRLAKKYEATLEKCCAEANPPACYGTVLAEFQPLVEEPKNLVKTNCDLYEKLGEYGFQNAILVRYTQKAPQVSTPTLVEAARNLGRVGTKCCTLPEDQRLPCVEDYLSAILNRVCLLHEKTPVSEHVTKCCSGSLVERRPCFSALTVDETYVPKEFKAETFTFHSDICTL

SEQ ID NO: 71 - DNA, 3456 bp, Artificial Sequence
  ENPP121-Fc nucleotide sequence
atggaaagggacggatgcgccggtggtggatctcgcggaggcgaaggtggaagggcccctagggaaggacctgccggaaacggaagggacaggggacgctctcacgccgctgaagctccaggcgaccctcaggccgctgcctctctgctggctcctatggacgtcggagaagaacccctggaaaaggccgccagggccaggactgccaaggaccccaacacctacaagatcatctccctcttcactttcgccgtcggagtcaacatctgcctgggattcaccgccggactgaagcccagctgcgccaaagaagtgaagtcctgcaagggccggtgcttcgagcggaccttcggcaactgcagatgcgacgccgcctgtgtggaactgggcaactgctgcctggactaccaggaaacctgcatcgagcccgagcacatctggacctgcaacaagttcagatgcggcgagaagcggctgaccagatccctgtgtgcctgcagcgacgactgcaaggacaagggcgactgctgcatcaactacagcagcgtgtgccagggcgagaagtcctgggtggaagaaccctgcgagagcatcaacgagccccagtgccctgccggcttcgagacacctcctaccctgctgttcagcctggacggctttcgggccgagtacctgcacacatggggaggcctgctgcccgtgatcagcaagctgaagaagtgcggcacctacaccaagaacatgcggcccgtgtaccccaccaagaccttccccaaccactactccatcgtgaccggcctgtaccccgagagccacggcatcatcgacaacaagatgtacgaccccaagatgaacgccagcttcagcctgaagtccaaagagaagttcaaccccgagtggtataagggcgagcccatctgggtcaccgccaagtaccagggcctgaaaagcggcacattcttttggcccggcagcgacgtggaaatcaacggcatcttccccgacatctataagatgtacaacggcagcgtgcccttcgaggaacggatcctggctgtgctgcagtggctgcagctgcccaaggatgagcggccccacttctacaccctgtacctggaagaacctgacagcagcggccacagctacggccctgtgtccagcgaagtgatcaaggccctgcagcgggtggacggcatggtgggaatgctgatggacggcctgaaagagctgaacctgcacagatgcctgaacctgatcctgatcagcgaccacggcatggaacagggatcctgcaagaagtacatctacctgaacaagtacctgggcgacgtgaagaacatcaaagtgatctacggcccagccgccagactgaggcctagcgacgtgcccgacaagtactacagcttcaactacgagggaatcgcccggaacctgagctgcagagagcccaaccagcacttcaagccctacctgaagcacttcctgcccaagcggctgcacttcgccaagagcgacagaatcgagcccctgaccttctacctggacccccagtggcagctggccctgaatcccagcgagagaaagtactgcggcagcggcttccacggctccgacaacgtgttcagcaacatgcaggccctgttcgtgggctacggacccggctttaagcacggcatcgaggccgacaccttcgagaacatcgaggtgtacaatctgatgtgcgacctgctgaatctgacccctgcccccaacaatggcacccacggcagcctgaaccatctgctgaagaaccccgtgtacacccctaagcaccccaaagaggtgcaccccctggtgcagtgccccttcaccagaaaccccagagacaacctgggctgtagctgcaaccccagcatcctgcccatcgaggacttccagacccagttcaacctgaccgtggccgaggaaaagatcatcaagcacgagacactgccctacggcagaccccgggtgctgcagaaagagaacaccatctgcctgctgagccagcaccagttcatgagcggctactcccaggacatcctgatgcccctgtggaccagctacaccgtggaccggaacgacagcttctccaccgaggatttcagcaactgcctgtaccaggatttccggatccccctgagccccgtgcacaagtgcagcttctacaagaacaacaccaaggtgtcctacggcttcctgagccctccccagctgaacaagaacagctccggcatctacagcgaggccctgctgactaccaacatcgtgcccatgtaccagagcttccaagtgatctggcggtacttccacgacaccctgctgcggaagtacgccgaagaacggaacggcgtgaacgtggtgtccggcccagtgttcgacttcgactacgacggcagatgtgacagcctggaaaatctgcggcagaaaagaagagtgatccggaaccaggaaattctgatccctacccacttctttatcgtgctgacaagctgcaaggataccagccagacccccctgcactgcgagaacctggataccctggccttcatcctgcctcaccggaccgacaacagcgagagctgtgtgcacggcaagcacgacagctcttgggtggaagaactgctgatgctgcaccgggccagaatcaccgatgtggaacacatcaccggcctgagcttttaccagcagcggaaagaacccgtgtccgatatcctgaagctgaaaacccatctgcccaccttcagccaggaagatgacaagacccacacttgccccccctgcccagctcctgaactgctgggaggaccctctgtgttcctgttccccccaaagcccaaggacaccctgatgatctctaggacccccgaagtcacttgcgtcgtcgtcgacgtgtcccacgaggaccctgaagtcaagttcaactggtacgtcgacggtgtcgaagtccacaacgccaagaccaagcccagggaagaacagtacaactctacctaccgcgtcgtcagcgtcctgaccgtcctgcaccaggactggctgaacggaaaggaatacaagtgcaaggtgtccaacaaggccctgcctgcccccatcgaaaagaccatctctaaggccaagggacagccccgcgaaccccaggtctacaccctgccaccctctagggaagaaatgaccaagaaccaggtgtccctgacctgcctggtcaagggattctacccctctgacatcgccgtcgaatgggaatctaacggacagcccgaaaacaactacaagaccaccccccctgtcctggactctgacggatcattcttcctgtactctaagctgactgtcgacaagtctaggtggcagcagggaaacgtgttctcttgctctgtcatgcacgaagccctgcacaaccactacacccagaagtctctgtctctgtcccccggaaag

SEQ ID NO: 72 - DNA, 4662 bp, Artificial Sequence
  ENPP121-Albumin nucleotide sequence
atggaaagggacggatgcgccggtggtggatctcgcggaggcgaaggtggaagggcccctagggaaggacctgccggaaacggaagggacaggggacgctctcacgccgctgaagctccaggcgaccctcaggccgctgcctctctgctggctcctatggacgtcggagaagaacccctggaaaaggccgccagggccaggactgccaaggaccccaacacctacaagatcatctccctcttcactttcgccgtcggagtcaacatctgcctgggattcaccgccggactgaagcccagctgcgccaaagaagtgaagtcctgcaagggccggtgcttcgagcggaccttcggcaactgcagatgcgacgccgcctgtgtggaactgggcaactgctgcctggactaccaggaaacctgcatcgagcccgagcacatctggacctgcaacaagttcagatgcggcgagaagcggctgaccagatccctgtgtgcctgcagcgacgactgcaaggacaagggcgactgctgcatcaactacagcagcgtgtgccagggcgagaagtcctgggtggaagaaccctgcgagagcatcaacgagccccagtgccctgccggcttcgagacacctcctaccctgctgttcagcctggacggctttcgggccgagtacctgcacacatggggaggcctgctgcccgtgatcagcaagctgaagaagtgcggcacctacaccaagaacatgcggcccgtgtaccccaccaagaccttccccaaccactactccatcgtgaccggcctgtaccccgagagccacggcatcatcgacaacaagatgtacgaccccaagatgaacgccagcttcagcctgaagtccaaagagaagttcaaccccgagtggtataagggcgagcccatctgggtcaccgccaagtaccagggcctgaaaagcggcacattcttttggcccggcagcgacgtggaaatcaacggcatcttccccgacatctataagatgtacaacggcagcgtgcccttcgaggaacggatcctggctgtgctgcagtggctgcagctgcccaaggatgagcggccccacttctacaccctgtacctggaagaacctgacagcagcggccacagctacggccctgtgtccagcgaagtgatcaaggccctgcagcgggtggacggcatggtgggaatgctgatggacggcctgaaagagctgaacctgcacagatgcctgaacctgatcctgatcagcgaccacggcatggaacagggatcctgcaagaagtacatctacctgaacaagtacctgggcgacgtgaagaacatcaaagtgatctacggcccagccgccagactgaggcctagcgacgtgcccgacaagtactacagcttcaactacgagggaatcgcccggaacctgagctgcagagagcccaaccagcacttcaagccctacctgaagcacttcctgcccaagcggctgcacttcgccaagagcgacagaatcgagcccctgaccttctacctggacccccagtggcagctggccctgaatcccagcgagagaaagtactgcggcagcggcttccacggctccgacaacgtgttcagcaacatgcaggccctgttcgtgggctacggacccggctttaagcacggcatcgaggccgacaccttcgagaacatcgaggtgtacaatctgatgtgcgacctgctgaatctgacccctgcccccaacaatggcacccacggcagcctgaaccatctgctgaagaaccccgtgtacacccctaagcaccccaaagaggtgcaccccctggtgcagtgccccttcaccagaaaccccagagacaacctgggctgtagctgcaaccccagcatcctgcccatcgaggacttccagacccagttcaacctgaccgtggccgaggaaaagatcatcaagcacgagacactgccctacggcagaccccgggtgctgcagaaagagaacaccatctgcctgctgagccagcaccagttcatgagcggctactcccaggacatcctgatgcccctgtggaccagctacaccgtggaccggaacgacagcttctccaccgaggatttcagcaactgcctgtaccaggatttccggatccccctgagccccgtgcacaagtgcagcttctacaagaacaacaccaaggtgtcctacggcttcctgagccctccccagctgaacaagaacagctccggcatctacagcgaggccctgctgactaccaacatcgtgcccatgtaccagagcttccaagtgatctggcggtacttccacgacaccctgctgcggaagtacgccgaagaacggaacggcgtgaacgtggtgtccggcccagtgttcgacttcgactacgacggcagatgtgacagcctggaaaatctgcggcagaaaagaagagtgatccggaaccaggaaattctgatccctacccacttctttatcgtgctgacaagctgcaaggataccagccagacccccctgcactgcgagaacctggataccctggccttcatcctgcctcaccggaccgacaacagcgagagctgtgtgcacggcaagcacgacagctcttgggtggaagaactgctgatgctgcaccgggccagaatcaccgatgtggaacacatcaccggcctgagcttttaccagcagcggaaagaacccgtgtccgatatcctgaagctgaaaacccatctgcccaccttcagccaggaagatggtggaggaggctctggtggaggcggtagcggaggcggagggtcgggaggttctggatcaatgaagtgggtaacctttatttcccttctttttctctttagctcggcttattccaggggtgtgtttcgtcgagatgcacacaagagtgaggttgctcatcggtttaaagatttgggagaagaaaatttcaaagccttggtgttgattgcctttgctcagtatcttcagcagtgtccatttgaagatcatgtaaaattagtgaatgaagtaactgaatttgcaaaaacatgtgttgctgatgagtcagctgaaaattgtgacaaatcacttcataccctttttggagacaaattatgcacagttgcaactcttcgtgaaacctatggtgaaatggctgactgctgtgcaaaacaagaacctgagagaaatgaatgcttcttgcaacacaaagatgacaacccaaacctcccccgattggtgagaccagaggttgatgtgatgtgcactgcttttcatgacaatgaagagacatttttgaaaaaatacttatatgaaattgccagaagacatccttacttttatgccccggaactccttttctttgctaaaaggtataaagctgcttttacagaatgttgccaagctgctgataaagctgcctgcctgttgccaaagctcgatgaacttcgggatgaagggaaggcttcgtctgccaaacagagactcaagtgtgccagtctccaaaaatttggagaaagagctttcaaagcatgggcagtagctcgcctgagccagagatttcccaaagctgagtttgcagaagtttccaagttagtgacagatcttaccaaagtccacacggaatgctgccatggagatctgcttgaatgtgctgatgacagggcggaccttgccaagtatatctgtgaaaatcaagattcgatctccagtaaactgaaggaatgctgtgaaaaacctctgttggaaaaatcccactgcattgccgaagtggaaaatgatgagatgcctgctgacttgccttcattagctgctgattttgttgaaagtaaggatgtttgcaaaaactatgctgaggcaaaggatgtcttcctgggcatgtttttgtatgaatatgcaagaaggcatcctgattactctgtcgtgctgctgctgagacttgccaagacatatgaaaccactctagagaagtgctgtgccgctgcagatcctcatgaatgctatgccaaagtgttcgatgaatttaaacctcttgtggaagagcctcagaatttaatcaaacaaaattgtgagctttttgagcagcttggagagtacaaattccagaatgcgctattagttcgttacaccaagaaagtaccccaagtgtcaactccaactcttgtagaggtctcaagaaacctaggaaaagtgggcagcaaatgttgtaaacatcctgaagcaaaaagaatgccctgtgcagaagactatctatccgtggtcctgaaccagttatgtgtgttgcatgagaaaacgccagtaagtgacagagtcaccaaatgctgcacagaatccttggtgaacaggcgaccatgcttttcagctctggaagtcgatgaaacatacgttcccaaagagtttaatgctgaaacattcaccttccatgcagatatatgcacactttctgagaaggagagacaaatcaagaaacaaactgcacttgttgagctcgtgaaacacaagcccaaggcaacaaaagagcaactgaaagctgttatggatgatttcgcagcttttgtagagaagtgctgcaaggctgacgataaggagacctgctttgccgaggagggtaaaaaacttgttgctgcaagtcaagctgccttaggctta

SEQ ID NO: 73 - DNA, 3228 bp, Artificial Sequence
  ENPP7-1-Fc nucleotide sequence
atgagaggacctgccgtcctgctgaccgtcgccctggctaccttgctggcccctggtgctggtgcacccagctgcgccaaagaagtgaagtcctgcaagggccggtgcttcgagcggaccttcggcaactgcagatgcgacgccgcctgtgtggaactgggcaactgctgcctggactaccaggaaacctgcatcgagcccgagcacatctggacctgcaacaagttcagatgcggcgagaagcggctgaccagatccctgtgtgcctgcagcgacgactgcaaggacaagggcgactgctgcatcaactacagcagcgtgtgccagggcgagaagtcctgggtggaagaaccctgcgagagcatcaacgagccccagtgccctgccggcttcgagacacctcctaccctgctgttcagcctggacggctttcgggccgagtacctgcacacatggggaggcctgctgcccgtgatcagcaagctgaagaagtgcggcacctacaccaagaacatgcggcccgtgtaccccaccaagaccttccccaaccactactccatcgtgaccggcctgtaccccgagagccacggcatcatcgacaacaagatgtacgaccccaagatgaacgccagcttcagcctgaagtccaaagagaagttcaaccccgagtggtataagggcgagcccatctgggtcaccgccaagtaccagggcctgaaaagcggcacattcttttggcccggcagcgacgtggaaatcaacggcatcttccccgacatctataagatgtacaacggcagcgtgcccttcgaggaacggatcctggctgtgctgcagtggctgcagctgcccaaggatgagcggccccacttctacaccctgtacctggaagaacctgacagcagcggccacagctacggccctgtgtccagcgaagtgatcaaggccctgcagcgggtggacggcatggtgggaatgctgatggacggcctgaaagagctgaacctgcacagatgcctgaacctgatcctgatcagcgaccacggcatggaacagggatcctgcaagaagtacatctacctgaacaagtacctgggcgacgtgaagaacatcaaagtgatctacggcccagccgccagactgaggcctagcgacgtgcccgacaagtactacagcttcaactacgagggaatcgcccggaacctgagctgcagagagcccaaccagcacttcaagccctacctgaagcacttcctgcccaagcggctgcacttcgccaagagcgacagaatcgagcccctgaccttctacctggacccccagtggcagctggccctgaatcccagcgagagaaagtactgcggcagcggcttccacggctccgacaacgtgttcagcaacatgcaggccctgttcgtgggctacggacccggctttaagcacggcatcgaggccgacaccttcgagaacatcgaggtgtacaatctgatgtgcgacctgctgaatctgacccctgcccccaacaatggcacccacggcagcctgaaccatctgctgaagaaccccgtgtacacccctaagcaccccaaagaggtgcaccccctggtgcagtgccccttcaccagaaaccccagagacaacctgggctgtagctgcaaccccagcatcctgcccatcgaggacttccagacccagttcaacctgaccgtggccgaggaaaagatcatcaagcacgagacactgccctacggcagaccccgggtgctgcagaaagagaacaccatctgcctgctgagccagcaccagttcatgagcggctactcccaggacatcctgatgcccctgtggaccagctacaccgtggaccggaacgacagcttctccaccgaggatttcagcaactgcctgtaccaggatttccggatccccctgagccccgtgcacaagtgcagcttctacaagaacaacaccaaggtgtcctacggcttcctgagccctccccagctgaacaagaacagctccggcatctacagcgaggccctgctgactaccaacatcgtgcccatgtaccagagcttccaagtgatctggcggtacttccacgacaccctgctgcggaagtacgccgaagaacggaacggcgtgaacgtggtgtccggcccagtgttcgacttcgactacgacggcagatgtgacagcctggaaaatctgcggcagaaaagaagagtgatccggaaccaggaaattctgatccctacccacttctttatcgtgctgacaagctgcaaggataccagccagacccccctgcactgcgagaacctggataccctggccttcatcctgcctcaccggaccgacaacagcgagagctgtgtgcacggcaagcacgacagctcttgggtggaagaactgctgatgctgcaccgggccagaatcaccgatgtggaacacatcaccggcctgagcttttaccagcagcggaaagaacccgtgtccgatatcctgaagctgaaaacccatctgcccaccttcagccaggaagatgacaagacccacacttgccccccctgcccagctcctgaactgctgggaggaccctctgtgttcctgttccccccaaagcccaaggacaccctgatgatctctaggacccccgaagtcacttgcgtcgtcgtcgacgtgtcccacgaggaccctgaagtcaagttcaactggtacgtcgacggtgtcgaagtccacaacgccaagaccaagcccagggaagaacagtacaactctacctaccgcgtcgtcagcgtcctgaccgtcctgcaccaggactggctgaacggaaaggaatacaagtgcaaggtgtccaacaaggccctgcctgcccccatcgaaaagaccatctctaaggccaagggacagccccgcgaaccccaggtctacaccctgccaccctctagggaagaaatgaccaagaaccaggtgtccctgacctgcctggtcaagggattctacccctctgacatcgccgtcgaatgggaatctaacggacagcccgaaaacaactacaagaccaccccccctgtcctggactctgacggatcattcttcctgtactctaagctgactgtcgacaagtctaggtggcagcagggaaacgtgttctcttgctctgtcatgcacgaagccctgcacaaccactacacccagaagtctctgtctctgtcccccggaaag

SEQ ID NO: 74 - DNA, 4434 bp, Artificial Sequence
  ENPP7-NPP1-Albumin nucleotide sequence
atgagaggacctgccgtcctgctgaccgtcgccctggctaccttgctggcccctggtgctggtgcacccagctgcgccaaagaagtgaagtcctgcaagggccggtgcttcgagcggaccttcggcaactgcagatgcgacgccgcctgtgtggaactgggcaactgctgcctggactaccaggaaacctgcatcgagcccgagcacatctggacctgcaacaagttcagatgcggcgagaagcggctgaccagatccctgtgtgcctgcagcgacgactgcaaggacaagggcgactgctgcatcaactacagcagcgtgtgccagggcgagaagtcctgggtggaagaaccctgcgagagcatcaacgagccccagtgccctgccggcttcgagacacctcctaccctgctgttcagcctggacggctttcgggccgagtacctgcacacatggggaggcctgctgcccgtgatcagcaagctgaagaagtgcggcacctacaccaagaacatgcggcccgtgtaccccaccaagaccttccccaaccactactccatcgtgaccggcctgtaccccgagagccacggcatcatcgacaacaagatgtacgaccccaagatgaacgccagcttcagcctgaagtccaaagagaagttcaaccccgagtggtataagggcgagcccatctgggtcaccgccaagtaccagggcctgaaaagcggcacattcttttggcccggcagcgacgtggaaatcaacggcatcttccccgacatctataagatgtacaacggcagcgtgcccttcgaggaacggatcctggctgtgctgcagtggctgcagctgcccaaggatgagcggccccacttctacaccctgtacctggaagaacctgacagcagcggccacagctacggccctgtgtccagcgaagtgatcaaggccctgcagcgggtggacggcatggtgggaatgctgatggacggcctgaaagagctgaacctgcacagatgcctgaacctgatcctgatcagcgaccacggcatggaacagggatcctgcaagaagtacatctacctgaacaagtacctgggcgacgtgaagaacatcaaagtgatctacggcccagccgccagactgaggcctagcgacgtgcccgacaagtactacagcttcaactacgagggaatcgcccggaacctgagctgcagagagcccaaccagcacttcaagccctacctgaagcacttcctgcccaagcggctgcacttcgccaagagcgacagaatcgagcccctgaccttctacctggacccccagtggcagctggccctgaatcccagcgagagaaagtactgcggcagcggcttccacggctccgacaacgtgttcagcaacatgcaggccctgttcgtgggctacggacccggctttaagcacggcatcgaggccgacaccttcgagaacatcgaggtgtacaatctgatgtgcgacctgctgaatctgacccctgcccccaacaatggcacccacggcagcctgaaccatctgctgaagaaccccgtgtacacccctaagcaccccaaagaggtgcaccccctggtgcagtgccccttcaccagaaaccccagagacaacctgggctgtagctgcaaccccagcatcctgcccatcgaggacttccagacccagttcaacctgaccgtggccgaggaaaagatcatcaagcacgagacactgccctacggcagaccccgggtgctgcagaaagagaacaccatctgcctgctgagccagcaccagttcatgagcggctactcccaggacatcctgatgcccctgtggaccagctacaccgtggaccggaacgacagcttctccaccgaggatttcagcaactgcctgtaccaggatttccggatccccctgagccccgtgcacaagtgcagcttctacaagaacaacaccaaggtgtcctacggcttcctgagccctccccagctgaacaagaacagctccggcatctacagcgaggccctgctgactaccaacatcgtgcccatgtaccagagcttccaagtgatctggcggtacttccacgacaccctgctgcggaagtacgccgaagaacggaacggcgtgaacgtggtgtccggcccagtgttcgacttcgactacgacggcagatgtgacagcctggaaaatctgcggcagaaaagaagagtgatccggaaccaggaaattctgatccctacccacttctttatcgtgctgacaagctgcaaggataccagccagacccccctgcactgcgagaacctggataccctggccttcatcctgcctcaccggaccgacaacagcgagagctgtgtgcacggcaagcacgacagctcttgggtggaagaactgctgatgctgcaccgggccagaatcaccgatgtggaacacatcaccggcctgagcttttaccagcagcggaaagaacccgtgtccgatatcctgaagctgaaaacccatctgcccaccttcagccaggaagatggtggaggaggctctggtggaggcggtagcggaggcggagggtcgggaggttctggatcaatgaagtgggtaacctttatttcccttctttttctctttagctcggcttattccaggggtgtgtttcgtcgagatgcacacaagagtgaggttgctcatcggtttaaagatttgggagaagaaaatttcaaagccttggtgttgattgcctttgctcagtatcttcagcagtgtccatttgaagatcatgtaaaattagtgaatgaagtaactgaatttgcaaaaacatgtgttgctgatgagtcagctgaaaattgtgacaaatcacttcataccctttttggagacaaattatgcacagttgcaactcttcgtgaaacctatggtgaaatggctgactgctgtgcaaaacaagaacctgagagaaatgaatgcttcttgcaacacaaagatgacaacccaaacctcccccgattggtgagaccagaggttgatgtgatgtgcactgcttttcatgacaatgaagagacatttttgaaaaaatacttatatgaaattgccagaagacatccttacttttatgccccggaactccttttctttgctaaaaggtataaagctgcttttacagaatgttgccaagctgctgataaagctgcctgcctgttgccaaagctcgatgaacttcgggatgaagggaaggcttcgtctgccaaacagagactcaagtgtgccagtctccaaaaatttggagaaagagctttcaaagcatgggcagtagctcgcctgagccagagatttcccaaagctgagtttgcagaagtttccaagttagtgacagatcttaccaaagtccacacggaatgctgccatggagatctgcttgaatgtgctgatgacagggcggaccttgccaagtatatctgtgaaaatcaagattcgatctccagtaaactgaaggaatgctgtgaaaaacctctgttggaaaaatcccactgcattgccgaagtggaaaatgatgagatgcctgctgacttgccttcattagctgctgattttgttgaaagtaaggatgtttgcaaaaactatgctgaggcaaaggatgtcttcctgggcatgtttttgtatgaatatgcaagaaggcatcctgattactctgtcgtgctgctgctgagacttgccaagacatatgaaaccactctagagaagtgctgtgccgctgcagatcctcatgaatgctatgccaaagtgttcgatgaatttaaacctcttgtggaagagcctcagaatttaatcaaacaaaattgtgagctttttgagcagcttggagagtacaaattccagaatgcgctattagttcgttacaccaagaaagtaccccaagtgtcaactccaactcttgtagaggtctcaagaaacctaggaaaagtgggcagcaaatgttgtaaacatcctgaagcaaaaagaatgccctgtgcagaagactatctatccgtggtcctgaaccagttatgtgtgttgcatgagaaaacgccagtaagtgacagagtcaccaaatgctgcacagaatccttggtgaacaggcgaccatgcttttcagctctggaagtcgatgaaacatacgttcccaaagagtttaatgctgaaacattcaccttccatgcagatatatgcacactttctgagaaggagagacaaatcaagaaacaaactgcacttgttgagctcgtgaaacacaagcccaaggcaacaaaagagcaactgaaagctgttatggatgatttcgcagcttttgtagagaagtgctgcaaggctgacgataaggagacctgctttgccgaggagggtaaaaaacttgttgctgcaagtcaagctgccttaggctta

SEQ ID NO: 75 - DNA, 2625 bp, Artificial Sequence
  ENPP3 nucleotide sequence
atggaatctacgttgactttagcaacggaacaacctgttaagaagaacactcttaagaaatataaaatagcttgcattgttcttcttgctttgctggtgatcatgtcacttggattaggcctggggcttggactcaggaaactggaaaagcaaggcagctgcaggaagaagtgctttgatgcatcatttagaggactggagaactgccggtgtgatgtggcatgtaaagaccgaggtgattgctgctgggattttgaagacacctgtgtggaatcaactcgaatatggatgtgcaataaatttcgttgtggagagaccagattagaggccagcctttgctcttgttcagatgactgtttgcagaggaaagattgctgtgctgactataagagtgtttgccaaggagaaacctcatggctggaagaaaactgtgacacagcccagcagtctcagtgcccagaagggtttgacctgccaccagttatcttgttttctatggatggatttagagctgaatatttatacacatgggatactttaatgccaaatatcaataaactgaaaacatgtggaattcattcaaaatacatgagagctatgtatcctaccaaaaccttcccaaatcattacaccattgtcacgggcttgtatccagagtcacatggcatcattgacaataatatgtatgatgtaaatctcaacaagaatttttcactttcttcaaaggaacaaaataatccagcctggtggcatgggcaaccaatgtggctgacagcaatgtatcaaggtttaaaagccgctacctacttttggcccggatcagaagtggctataaatggctcctttccttccatatacatgccttacaacggaagtgtcccatttgaagagaggatttctacactgttaaaatggctggacctgcccaaagctgaaagacccaggttttataccatgtattttgaagaacctgattcctctggacatgcaggtggaccagtcagtgccagagtaattaaagccttacaggtagtagatcatgcttttgggatgttgatggaaggcctgaagcagcggaatttgcacaactgtgtcaatatcatccttctggctgaccatggaatggaccagacttattgtaacaagatggaatacatgactgattattttcccagaataaacttcttctacatgtacgaagggcctgccccccgcatccgagctcataatatacctcatgacttttttagttttaattctgaggaaattgttagaaacctcagttgccgaaaacctgatcagcatttcaagccctatttgactcctgatttgccaaagcgactgcactatgccaagaacgtcagaatcgacaaagttcatctctttgtggatcaacagtggctggctgttaggagtaaatcaaatacaaattgtggaggaggcaaccatggttataacaatgagtttaggagcatggaggctatctttctggcacatggacccagttttaaagagaagactgaagttgaaccatttgaaaatattgaagtctataacctaatgtgtgatcttctacgcattcaaccagcaccaaacaatggaacccatggtagtttaaaccatcttctgaaggtgcctttttatgagccatcccatgcagaggaggtgtcaaagttttctgtttgtggctttgctaatccattgcccacagagtctcttgactgtttctgccctcacctacaaaatagtactcagctggaacaagtgaatcagatgctaaatctcacccaagaagaaataacagcaacagtgaaagtaaatttgccatttgggaggcctagggtactgcagaagaacgtggaccactgtctcctttaccacagggaatatgtcagtggatttggaaaagctatgaggatgcccatgtggagttcatacacagtcccccagttgggagacacatcgcctctgcctcccactgtcccagactgtctgcgggctgatgtcagggttcctccttctgagagccaaaaatgttccttctatttagcagacaagaatatcacccacggcttcctctatcctcctgccagcaatagaacatcagatagccaatatgatgctttaattactagcaatttggtacctatgtatgaagaattcagaaaaatgtgggactacttccacagtgttcttcttataaaacatgccacagaaagaaatggagtaaatgtggttagtggaccaatatttgattataattatgatggccattttgatgctccagatgaaattaccaaacatttagccaacactgatgttcccatcccaacacactactttgtggtgctgaccagttgtaaaaacaagagccacacaccggaaaactgccctgggtggctggatgtcctaccctttatcatccctcaccgacctaccaacgtggagagctgtcctgaaggtaaaccagaagctctttgggttgaagaaagatttacagctcacattgcccgggtccgtgatgtagaacttctcactgggcttgacttctatcaggataaagtgcagcctgtctctgaaattttgcaactaaagacatatttaccaacatttgaaaccactatt

SEQ ID NO: 76 - DNA, 2775 bp, Artificial Sequence
  ENPP1 nucleotide sequence
atggaacgggacggctgtgccggcggaggatcaagaggcggagaaggcggcagagcccctagagaaggacctgccggcaacggcagagacagaggcagatctcatgccgccgaagcccctggcgatcctcaggctgctgcttctctgctggcccccatggatgtgggcgaggaacctctggaaaaggccgccagagccagaaccgccaaggaccccaacacctacaaggtgctgagcctggtgctgtccgtgtgcgtgctgaccaccatcctgggctgcatcttcggcctgaagcccagctgcgccaaagaagtgaagtcctgcaagggccggtgcttcgagcggaccttcggcaactgcagatgcgacgccgcctgtgtggaactgggcaactgctgcctggactaccaggaaacctgcatcgagcccgagcacatctggacctgcaacaagttcagatgcggcgagaagcggctgaccagatccctgtgtgcctgcagcgacgactgcaaggacaagggcgactgctgcatcaactacagcagcgtgtgccagggcgagaagtcctgggtggaagaaccctgcgagagcatcaacgagccccagtgccctgccggcttcgagacacctcctaccctgctgttcagcctggacggctttcgggccgagtacctgcacacatggggaggcctgctgcccgtgatcagcaagctgaagaagtgcggcacctacaccaagaacatgcggcccgtgtaccccaccaagaccttccccaaccactactccatcgtgaccggcctgtaccccgagagccacggcatcatcgacaacaagatgtacgaccccaagatgaacgccagcttcagcctgaagtccaaagagaagttcaaccccgagtggtataagggcgagcccatctgggtcaccgccaagtaccagggcctgaaaagcggcacattcttttggcccggcagcgacgtggaaatcaacggcatcttccccgacatctataagatgtacaacggcagcgtgcccttcgaggaacggatcctggctgtgctgcagtggctgcagctgcccaaggatgagcggccccacttctacaccctgtacctggaagaacctgacagcagcggccacagctacggccctgtgtccagcgaagtgatcaaggccctgcagcgggtggacggcatggtgggaatgctgatggacggcctgaaagagctgaacctgcacagatgcctgaacctgatcctgatcagcgaccacggcatggaacagggatcctgcaagaagtacatctacctgaacaagtacctgggcgacgtgaagaacatcaaagtgatctacggcccagccgccagactgaggcctagcgacgtgcccgacaagtactacagcttcaactacgagggaatcgcccggaacctgagctgcagagagcccaaccagcacttcaagccctacctgaagcacttcctgcccaagcggctgcacttcgccaagagcgacagaatcgagcccctgaccttctacctggacccccagtggcagctggccctgaatcccagcgagagaaagtactgcggcagcggcttccacggctccgacaacgtgttcagcaacatgcaggccctgttcgtgggctacggacccggctttaagcacggcatcgaggccgacaccttcgagaacatcgaggtgtacaatctgatgtgcgacctgctgaatctgacccctgcccccaacaatggcacccacggcagcctgaaccatctgctgaagaaccccgtgtacacccctaagcaccccaaagaggtgcaccccctggtgcagtgccccttcaccagaaaccccagagacaacctgggctgtagctgcaaccccagcatcctgcccatcgaggacttccagacccagttcaacctgaccgtggccgaggaaaagatcatcaagcacgagacactgccctacggcagaccccgggtgctgcagaaagagaacaccatctgcctgctgagccagcaccagttcatgagcggctactcccaggacatcctgatgcccctgtggaccagctacaccgtggaccggaacgacagcttctccaccgaggatttcagcaactgcctgtaccaggatttccggatccccctgagccccgtgcacaagtgcagcttctacaagaacaacaccaaggtgtcctacggcttcctgagccctccccagctgaacaagaacagctccggcatctacagcgaggccctgctgactaccaacatcgtgcccatgtaccagagcttccaagtgatctggcggtacttccacgacaccctgctgcggaagtacgccgaagaacggaacggcgtgaacgtggtgtccggcccagtgttcgacttcgactacgacggcagatgtgacagcctggaaaatctgcggcagaaaagaagagtgatccggaaccaggaaattctgatccctacccacttctttatcgtgctgacaagctgcaaggataccagccagacccccctgcactgcgagaacctggataccctggccttcatcctgcctcaccggaccgacaacagcgagagctgtgtgcacggcaagcacgacagctcttgggtggaagaactgctgatgctgcaccgggccagaatcaccgatgtggaacacatcaccggcctgagcttttaccagcagcggaaagaacccgtgtccgatatcctgaagctgaaaacccatctgcccaccttcagccaggaagat